European Patent Specification EP 3 615 565 B1, published March 26, 2025. Title: TCR AND PEPTIDES. Applicant: Ospedale San Raffaele S.r.l Fondazione Centro San Raffaele. The sequence listing filed with the application follows.

SEQUENCE LISTING (299 sequences)

SEQ ID NO: 1 - protein, 5 aa, Artificial Sequence
  TCR (T-cell receptor) amino acid sequence, Donor HD1
KALYS

SEQ ID NO: 2 - protein, 7 aa, Artificial Sequence
  TCR amino acid sequence, Donor HD1
LLKGGEQ

SEQ ID NO: 3 - protein, 13 aa, Artificial Sequence
  TCR amino acid sequence, Donor HD1
CGTAWINDYKLSF

SEQ ID NO: 4 - protein, 132 aa, Artificial Sequence
  TCR amino acid sequence, Donor HD1
METLLKVLSGTLLWQLTWVRSQQPVQSPQAVILREGEDAVINCSSSKALYSVHWYRQKHGEAPVFLMILLKGGEQKGHEKISASFNEKKQQSSLYLTASQLSYSGTYFCGTAWINDYKLSFGAGTTVTVRAN

SEQ ID NO: 5 - protein, 272 aa, Artificial Sequence
  TCR amino acid sequence, Donor HD1
METLLKVLSGTLLWQLTWVRSQQPVQSPQAVILREGEDAVINCSSSKALYSVHWYRQKHGEAPVFLMILLKGGEQKGHEKISASFNEKKQQSSLYLTASQLSYSGTYFCGTAWINDYKLSFGAGTTVTVRANIQNPDPAVYQLRDSKSSDKSVCLFTDFDSQTNVSQSKDSDVYITDKTVLDMRSMDFKSNSAVAWSNKSDFACANAFNNSIIPEDTFFPSPESSCDVKLVEKSFETDTNLNFQNLSVIGFRILLLKVAGFNLLMTLRLWSS

SEQ ID NO: 6 - protein, 5 aa, Artificial Sequence
  TCR amino acid sequence, Donor HD1
SGHDY

SEQ ID NO: 7 - protein, 6 aa, Artificial Sequence
  TCR amino acid sequence, Donor HD1
FNNNVP

SEQ ID NO: 8 - protein, 16 aa, Artificial Sequence
  TCR amino acid sequence, Donor HD1
CASRKTGGYSNQPQHF

SEQ ID NO: 9 - protein, 136 aa, Artificial Sequence
  TCR amino acid sequence, Donor HD1
MGSWTLCCVSLCILVAKHTDAGVIQSPRHEVTEMGQEVTLRCKPISGHDYLFWYRQTMMRGLELLIYFNNNVPIDDSGMPEDRFSAKMPNASFSTLKIQPSEPRDSAVYFCASRKTGGYSNQPQHFGDGTRLSILE

SEQ ID NO: 10 - protein, 312 aa, Artificial Sequence
  TCR amino acid sequence, Donor HD1
MGSWTLCCVSLCILVAKHTDAGVIQSPRHEVTEMGQEVTLRCKPISGHDYLFWYRQTMMRGLELLIYFNNNVPIDDSGMPEDRFSAKMPNASFSTLKIQPSEPRDSAVYFCASRKTGGYSNQPQHFGDGTRLSILEDLNKVFPPEVAVFEPSEAEISHTQKATLVCLATGFFPDHVELSWWVNGKEVHSGVSTDPQPLKEQPALNDSRYCLSSRLRVSATFWQNPRNHFRCQVQFYGLSENDEWTQDRAKPVTQIVSAEAWGRADCGFTSVSYQQGVLSATILYEILLGKATLYAVLVSALVLMAMVKRKDF

SEQ ID NO: 11 - protein, 314 aa, Artificial Sequence
  TCR amino acid sequence, Donor HD1
MGSWTLCCVSLCILVAKHTDAGVIQSPRHEVTEMGQEVTLRCKPISGHDYLFWYRQTMMRGLELLIYFNNNVPIDDSGMPEDRFSAKMPNASFSTLKIQPSEPRDSAVYFCASRKTGGYSNQPQHFGDGTRLSILEDLKNVFPPEVAVFEPSEAEISHTQKATLVCLATGFYPDHVELSWWVNGKEVHSGVSTDPQPLKEQPALNDSRYCLSSRLRVSATFWQNPRNHFRCQVQFYGLSENDEWTQDRAKPVTQIVSAEAWGRADCGFTSESYQQGVLSATILYEILLGKATLYAVLVSALVLMAMVKRKDSRG

SEQ ID NO: 12 - protein, 6 aa, Artificial Sequence
  TCR amino acid sequence, Donor HD2
SSVPPY

SEQ ID NO: 13 - protein, 8 aa, Artificial Sequence
  TCR amino acid sequence, Donor HD2
YTSAATLV

SEQ ID NO: 14 - protein, 14 aa, Artificial Sequence
  TCR amino acid sequence, Donor HD2
CAVRLSGSARQLTF

SEQ ID NO: 15 - protein, 134 aa, Artificial Sequence
  TCR amino acid sequence, Donor HD2
MLLLLVPVLEVIFTLGGTRAQSVTQLGSHVSVSEGALVLLRCNYSSSVPPYLFWYVQYPNQGLQLLLKYTSAATLVKGINGFEAEFKKSETSFHLTKPSAHMSDAAEYFCAVRLSGSARQLTFGSGTQLTVLPD

SEQ ID NO: 16 - protein, 274 aa, Artificial Sequence
  TCR amino acid sequence, Donor HD2
MLLLLVPVLEVIFTLGGTRAQSVTQLGSHVSVSEGALVLLRCNYSSSVPPYLFWYVQYPNQGLQLLLKYTSAATLVKGINGFEAEFKKSETSFHLTKPSAHMSDAAEYFCAVRLSGSARQLTFGSGTQLTVLPDIQNPDPAVYQLRDSKSSDKSVCLFTDFDSQTNVSQSKDSDVYITDKTVLDMRSMDFKSNSAVAWSNKSDFACANAFNNSIIPEDTFFPSPESSCDVKLVEKSFETDTNLNFQNLSVIGFRILLLKVAGFNLLMTLRLWSS

SEQ ID NO: 17 - protein, 7 aa, Artificial Sequence
  TCR amino acid sequence, Donor HD2
TSESDYY

SEQ ID NO: 18 - protein, 8 aa, Artificial Sequence
  TCR amino acid sequence, Donor HD2
QEAYKQQN

SEQ ID NO: 19 - protein, 14 aa, Artificial Sequence
  TCR amino acid sequence, Donor HD2
CAYRSLKYGNKLVF

SEQ ID NO: 20 - protein, 136 aa, Artificial Sequence
  TCR amino acid sequence, Donor HD2
MACPGFLWALVISTCLEFSMAQTVTQSQPEMSVQEAETVTLSCTYDTSESDYYLFWYKQPPSRQMILVIRQEAYKQQNATENRFSVNFQKAAKSFSLKISDSQLGDAAMYFCAYRSLKYGNKLVFGAGTILRVKSY

SEQ ID NO: 21 - protein, 276 aa, Artificial Sequence
  TCR amino acid sequence, Donor HD2
MACPGFLWALVISTCLEFSMAQTVTQSQPEMSVQEAETVTLSCTYDTSESDYYLFWYKQPPSRQMILVIRQEAYKQQNATENRFSVNFQKAAKSFSLKISDSQLGDAAMYFCAYRSLKYGNKLVFGAGTILRVKSYIQNPDPAVYQLRDSKSSDKSVCLFTDFDSQTNVSQSKDSDVYITDKTVLDMRSMDFKSNSAVAWSNKSDFACANAFNNSIIPEDTFFPSPESSCDVKLVEKSFETDTNLNFQNLSVIGFRILLLKVAGFNLLMTLRLWSS

SEQ ID NO: 22 - protein, 5 aa, Artificial Sequence
  TCR amino acid sequence, Donor HD2
SGHAT

SEQ ID NO: 23 - protein, 6 aa, Artificial Sequence
  TCR amino acid sequence, Donor HD2
FQNNGV

SEQ ID NO: 24 - protein, 12 aa, Artificial Sequence
  TCR amino acid sequence, Donor HD2
CASSLLGDEQYF

SEQ ID NO: 25 - protein, 132 aa, Artificial Sequence
  TCR amino acid sequence, Donor HD2
MGTRLLCWAALCLLGAELTEAGVAQSPRYKIIEKRQSVAFWCNPISGHATLYWYQQILGQGPKLLIQFQNNGVVDDSQLPKDRFSAERLKGVDSTLKIQPAKLEDSAVYLCASSLLGDEQYFGPGTRLTVTE

SEQ ID NO: 26 - protein, 308 aa, Artificial Sequence
  TCR amino acid sequence, Donor HD2
MGTRLLCWAALCLLGAELTEAGVAQSPRYKIIEKRQSVAFWCNPISGHATLYWYQQILGQGPKLLIQFQNNGVVDDSQLPKDRFSAERLKGVDSTLKIQPAKLEDSAVYLCASSLLGDEQYFGPGTRLTVTEDLNKVFPPEVAVFEPSEAEISHTQKATLVCLATGFFPDHVELSWWVNGKEVHSGVSTDPQPLKEQPALNDSRYCLSSRLRVSATFWQNPRNHFRCQVQFYGLSENDEWTQDRAKPVTQIVSAEAWGRADCGFTSVSYQQGVLSATILYEILLGKATLYAVLVSALVLMAMVKRKDF

SEQ ID NO: 27 - protein, 310 aa, Artificial Sequence
  TCR amino acid sequence, Donor HD2
MGTRLLCWAALCLLGAELTEAGVAQSPRYKIIEKRQSVAFWCNPISGHATLYWYQQILGQGPKLLIQFQNNGVVDDSQLPKDRFSAERLKGVDSTLKIQPAKLEDSAVYLCASSLLGDEQYFGPGTRLTVTEDLKNVFPPEVAVFEPSEAEISHTQKATLVCLATGFYPDHVELSWWVNGKEVHSGVSTDPQPLKEQPALNDSRYCLSSRLRVSATFWQNPRNHFRCQVQFYGLSENDEWTQDRAKPVTQIVSAEAWGRADCGFTSESYQQGVLSATILYEILLGKATLYAVLVSALVLMAMVKRKDSRG

SEQ ID NO: 28 - protein, 5 aa, Artificial Sequence
  TCR amino acid sequence, Donor HD2
SGHTA

SEQ ID NO: 29 - protein, 6 aa, Artificial Sequence
  TCR amino acid sequence, Donor HD2
FQGNSA

SEQ ID NO: 30 - protein, 16 aa, Artificial Sequence
  TCR amino acid sequence, Donor HD2
CASSLVALQGAGEQYF

SEQ ID NO: 31 - protein, 136 aa, Artificial Sequence
  TCR amino acid sequence, Donor HD2
MGTRLLFWVAFCLLGADHTGAGVSQSPSNKVTEKGKDVELRCDPISGHTALYWYRQSLGQGLEFLIYFQGNSAPDKSGLPSDRFSAERTGGSVSTLTIQRTQQEDSAVYLCASSLVALQGAGEQYFGPGTRLTVTE

SEQ ID NO: 32 - protein, 312 aa, Artificial Sequence
  TCR amino acid sequence, Donor HD2
MGTRLLFWVAFCLLGADHTGAGVSQSPSNKVTEKGKDVELRCDPISGHTALYWYRQSLGQGLEFLIYFQGNSAPDKSGLPSDRFSAERTGGSVSTLTIQRTQQEDSAVYLCASSLVALQGAGEQYFGPGTRLTVTEDLNKVFPPEVAVFEPSEAEISHTQKATLVCLATGFFPDHVELSWWVNGKEVHSGVSTDPQPLKEQPALNDSRYCLSSRLRVSATFWQNPRNHFRCQVQFYGLSENDEWTQDRAKPVTQIVSAEAWGRADCGFTSVSYQQGVLSATILYEILLGKATLYAVLVSALVLMAMVKRKDF

SEQ ID NO: 33 - protein, 314 aa, Artificial Sequence
  TCR amino acid sequence, Donor HD2
MGTRLLFWVAFCLLGADHTGAGVSQSPSNKVTEKGKDVELRCDPISGHTALYWYRQSLGQGLEFLIYFQGNSAPDKSGLPSDRFSAERTGGSVSTLTIQRTQQEDSAVYLCASSLVALQGAGEQYFGPGTRLTVTEDLKNVFPPEVAVFEPSEAEISHTQKATLVCLATGFYPDHVELSWWVNGKEVHSGVSTDPQPLKEQPALNDSRYCLSSRLRVSATFWQNPRNHFRCQVQFYGLSENDEWTQDRAKPVTQIVSAEAWGRADCGFTSESYQQGVLSATILYEILLGKATLYAVLVSALVLMAMVKRKDSRG

SEQ ID NO: 34 - protein, 6 aa, Artificial Sequence
  TCR amino acid sequence, Donor HD3
NSASQS

SEQ ID NO: 35 - protein, 6 aa, Artificial Sequence
  TCR amino acid sequence, Donor HD3
VYSSGN

SEQ ID NO: 36 - protein, 15 aa, Artificial Sequence
  TCR amino acid sequence, Donor HD3
CVVNLLSNQGGKLIF

SEQ ID NO: 37 - protein, 134 aa, Artificial Sequence
  TCR amino acid sequence, Donor HD3
MISLRVLLVILWLQLSWVWSQRKEVEQDPGPFNVPEGATVAFNCTYSNSASQSFFWYRQDCRKEPKLLMSVYSSGNEDGRFTAQLNRASQYISLLIRDSKLSDSATYLCVVNLLSNQGGKLIFGQGTELSVKPN

SEQ ID NO: 38 - protein, 274 aa, Artificial Sequence
  TCR amino acid sequence, Donor HD3
MISLRVLLVILWLQLSWVWSQRKEVEQDPGPFNVPEGATVAFNCTYSNSASQSFFWYRQDCRKEPKLLMSVYSSGNEDGRFTAQLNRASQYISLLIRDSKLSDSATYLCVVNLLSNQGGKLIFGQGTELSVKPNIQNPDPAVYQLRDSKSSDKSVCLFTDFDSQTNVSQSKDSDVYITDKTVLDMRSMDFKSNSAVAWSNKSDFACANAFNNSIIPEDTFFPSPESSCDVKLVEKSFETDTNLNFQNLSVIGFRILLLKVAGFNLLMTLRLWSS

SEQ ID NO: 39 - protein, 5 aa, Artificial Sequence
  TCR amino acid sequence, Donor HD3
LGHNA

SEQ ID NO: 40 - protein, 6 aa, Artificial Sequence
  TCR amino acid sequence, Donor HD3
YSLEER

SEQ ID NO: 41 - protein, 16 aa, Artificial Sequence
  TCR amino acid sequence, Donor HD3
CASSQDYLVSNEKLFF

SEQ ID NO: 42 - protein, 138 aa, Artificial Sequence
  TCR amino acid sequence, Donor HD3
MGCRLLCCAVLCLLGAGELVPMETGVTQTPRHLVMGMTNKKSLKCEQHLGHNAMYWYKQSAKKPLELMFVYSLEERVENNSVPSRFSPECPNSSHLFLHLHTLQPEDSALYLCASSQDYLVSNEKLFFGSGTQLSVLE

SEQ ID NO: 43 - protein, 314 aa, Artificial Sequence
  TCR amino acid sequence, Donor HD3
MGCRLLCCAVLCLLGAGELVPMETGVTQTPRHLVMGMTNKKSLKCEQHLGHNAMYWYKQSAKKPLELMFVYSLEERVENNSVPSRFSPECPNSSHLFLHLHTLQPEDSALYLCASSQDYLVSNEKLFFGSGTQLSVLEDLNKVFPPEVAVFEPSEAEISHTQKATLVCLATGFFPDHVELSWWVNGKEVHSGVSTDPQPLKEQPALNDSRYCLSSRLRVSATFWQNPRNHFRCQVQFYGLSENDEWTQDRAKPVTQIVSAEAWGRADCGFTSVSYQQGVLSATILYEILLGKATLYAVLVSALVLMAMVKRKDF

SEQ ID NO: 44 - protein, 316 aa, Artificial Sequence
  TCR amino acid sequence, Donor HD3
MGCRLLCCAVLCLLGAGELVPMETGVTQTPRHLVMGMTNKKSLKCEQHLGHNAMYWYKQSAKKPLELMFVYSLEERVENNSVPSRFSPECPNSSHLFLHLHTLQPEDSALYLCASSQDYLVSNEKLFFGSGTQLSVLEDLKNVFPPEVAVFEPSEAEISHTQKATLVCLATGFYPDHVELSWWVNGKEVHSGVSTDPQPLKEQPALNDSRYCLSSRLRVSATFWQNPRNHFRCQVQFYGLSENDEWTQDRAKPVTQIVSAEAWGRADCGFTSESYQQGVLSATILYEILLGKATLYAVLVSALVLMAMVKRKDSRG

SEQ ID NO: 45 - protein, 5 aa, Artificial Sequence
  TCR amino acid sequence, Donor HD4
TSINN

SEQ ID NO: 46 - protein, 7 aa, Artificial Sequence
  TCR amino acid sequence, Donor HD4
IRSNERE

SEQ ID NO: 47 - protein, 14 aa, Artificial Sequence
  TCR amino acid sequence, Donor HD4
CATDAYSGNTPLVF

SEQ ID NO: 48 - protein, 133 aa, Artificial Sequence
  TCR amino acid sequence, Donor HD4
METLLGVSLVILWLQLARVNSQQGEEDPQALSIQEGENATMNCSYKTSINNLQWYRQNSGRGLVHLILIRSNEREKHSGRLRVTLDTSKKSSSLLITASRAADTASYFCATDAYSGNTPLVFGKGTRLSVIAN

SEQ ID NO: 49 - protein, 273 aa, Artificial Sequence
  TCR amino acid sequence, Donor HD4
METLLGVSLVILWLQLARVNSQQGEEDPQALSIQEGENATMNCSYKTSINNLQWYRQNSGRGLVHLILIRSNEREKHSGRLRVTLDTSKKSSSLLITASRAADTASYFCATDAYSGNTPLVFGKGTRLSVIANIQNPDPAVYQLRDSKSSDKSVCLFTDFDSQTNVSQSKDSDVYITDKTVLDMRSMDFKSNSAVAWSNKSDFACANAFNNSIIPEDTFFPSPESSCDVKLVEKSFETDTNLNFQNLSVIGFRILLLKVAGFNLLMTLRLWSS

SEQ ID NO: 50 - protein, 6 aa, Artificial Sequence
  TCR amino acid sequence, Donor HD4
DSAIYN

SEQ ID NO: 51 - protein, 7 aa, Artificial Sequence
  TCR amino acid sequence, Donor HD4
IQSSQRE

SEQ ID NO: 52 - protein, 16 aa, Artificial Sequence
  TCR amino acid sequence, Donor HD4
CAVRAEIYNQGGKLIF

SEQ ID NO: 53 - protein, 135 aa, Artificial Sequence
  TCR amino acid sequence, Donor HD4
METLLGLLILWLQLQWVSSKQEVTQIPAALSVPEGENLVLNCSFTDSAIYNLQWFRQDPGKGLTSLLLIQSSQREQTSGRLNASLDKSSGRSTLYIAASQPGDSATYLCAVRAEIYNQGGKLIFGQGTELSVKPN

SEQ ID NO: 54 - protein, 275 aa, Artificial Sequence
  TCR amino acid sequence, Donor HD4
METLLGLLILWLQLQWVSSKQEVTQIPAALSVPEGENLVLNCSFTDSAIYNLQWFRQDPGKGLTSLLLIQSSQREQTSGRLNASLDKSSGRSTLYIAASQPGDSATYLCAVRAEIYNQGGKLIFGQGTELSVKPNIQNPDPAVYQLRDSKSSDKSVCLFTDFDSQTNVSQSKDSDVYITDKTVLDMRSMDFKSNSAVAWSNKSDFACANAFNNSIIPEDTFFPSPESSCDVKLVEKSFETDTNLNFQNLSVIGFRILLLKVAGFNLLMTLRLWSS

SEQ ID NO: 55 - protein, 5 aa, Artificial Sequence
  TCR amino acid sequence, Donor HD4
MNHNS

SEQ ID NO: 56 - protein, 6 aa, Artificial Sequence
  TCR amino acid sequence, Donor HD4
SASEGT

SEQ ID NO: 57 - protein, 14 aa, Artificial Sequence
  TCR amino acid sequence, Donor HD4
CASRAAGLDTEAFF

SEQ ID NO: 58 - protein, 133 aa, Artificial Sequence
  TCR amino acid sequence, Donor HD4
MSIGLLCCVAFSLLWASPVNAGVTQTPKFQVLKTGQSMTLQCAQDMNHNSMYWYRQDPGMGLRLIYYSASEGTTDKGEVPNGYNVSRLNKREFSLRLESAAPSQTSVYFCASRAAGLDTEAFFGQGTRLTVVE

SEQ ID NO: 59 - protein, 309 aa, Artificial Sequence
  TCR amino acid sequence, Donor HD4
MSIGLLCCVAFSLLWASPVNAGVTQTPKFQVLKTGQSMTLQCAQDMNHNSMYWYRQDPGMGLRLIYYSASEGTTDKGEVPNGYNVSRLNKREFSLRLESAAPSQTSVYFCASRAAGLDTEAFFGQGTRLTVVEDLNKVFPPEVAVFEPSEAEISHTQKATLVCLATGFFPDHVELSWWVNGKEVHSGVSTDPQPLKEQPALNDSRYCLSSRLRVSATFWQNPRNHFRCQVQFYGLSENDEWTQDRAKPVTQIVSAEAWGRADCGFTSVSYQQGVLSATILYEILLGKATLYAVLVSALVLMAMVKRKDF

SEQ ID NO: 60 - protein, 311 aa, Artificial Sequence
  TCR amino acid sequence, Donor HD4
MSIGLLCCVAFSLLWASPVNAGVTQTPKFQVLKTGQSMTLQCAQDMNHNSMYWYRQDPGMGLRLIYYSASEGTTDKGEVPNGYNVSRLNKREFSLRLESAAPSQTSVYFCASRAAGLDTEAFFGQGTRLTVVEDLKNVFPPEVAVFEPSEAEISHTQKATLVCLATGFYPDHVELSWWVNGKEVHSGVSTDPQPLKEQPALNDSRYCLSSRLRVSATFWQNPRNHFRCQVQFYGLSENDEWTQDRAKPVTQIVSAEAWGRADCGFTSESYQQGVLSATILYEILLGKATLYAVLVSALVLMAMVKRKDSRG

SEQ ID NO: 61 - protein, 5 aa, Artificial Sequence
  TCR amino acid sequence, Donor HD4
MNHNY

SEQ ID NO: 62 - protein, 6 aa, Artificial Sequence
  TCR amino acid sequence, Donor HD4
SVGAGI

SEQ ID NO: 63 - protein, 12 aa, Artificial Sequence
  TCR amino acid sequence, Donor HD4
CASTQTPYEQYF

SEQ ID NO: 64 - protein, 131 aa, Artificial Sequence
  TCR amino acid sequence, Donor HD4
MSISLLCCAAFPLLWAGPVNAGVTQTPKFRILKIGQSMTLQCTQDMNHNYMYWYRQDPGMGLKLIYYSVGAGITDKGEVPNGYNVSRSTTEDFPLRLELAAPSQTSVYFCASTQTPYEQYFGPGTRLTVTE

SEQ ID NO: 65 - protein, 307 aa, Artificial Sequence
  TCR amino acid sequence, Donor HD4
MSISLLCCAAFPLLWAGPVNAGVTQTPKFRILKIGQSMTLQCTQDMNHNYMYWYRQDPGMGLKLIYYSVGAGITDKGEVPNGYNVSRSTTEDFPLRLELAAPSQTSVYFCASTQTPYEQYFGPGTRLTVTEDLNKVFPPEVAVFEPSEAEISHTQKATLVCLATGFFPDHVELSWWVNGKEVHSGVSTDPQPLKEQPALNDSRYCLSSRLRVSATFWQNPRNHFRCQVQFYGLSENDEWTQDRAKPVTQIVSAEAWGRADCGFTSVSYQQGVLSATILYEILLGKATLYAVLVSALVLMAMVKRKDF

SEQ ID NO: 66 - protein, 309 aa, Artificial Sequence
  TCR amino acid sequence, Donor HD4
MSISLLCCAAFPLLWAGPVNAGVTQTPKFRILKIGQSMTLQCTQDMNHNYMYWYRQDPGMGLKLIYYSVGAGITDKGEVPNGYNVSRSTTEDFPLRLELAAPSQTSVYFCASTQTPYEQYFGPGTRLTVTEDLKNVFPPEVAVFEPSEAEISHTQKATLVCLATGFYPDHVELSWWVNGKEVHSGVSTDPQPLKEQPALNDSRYCLSSRLRVSATFWQNPRNHFRCQVQFYGLSENDEWTQDRAKPVTQIVSAEAWGRADCGFTSESYQQGVLSATILYEILLGKATLYAVLVSALVLMAMVKRKDSRG

SEQ ID NO: 67 - protein, 5 aa, Artificial Sequence
  TCR amino acid sequence, Donor HD4
SGHNS

SEQ ID NO: 68 - protein, 6 aa, Artificial Sequence
  TCR amino acid sequence, Donor HD4
FNNNVP

SEQ ID NO: 69 - protein, 15 aa, Artificial Sequence
  TCR amino acid sequence, Donor HD4
CASSTVGGEDYGYTF

SEQ ID NO: 70 - protein, 135 aa, Artificial Sequence
  TCR amino acid sequence, Donor HD4
MDSWTFCCVSLCILVAKHTDAGVIQSPRHEVTEMGQEVTLRCKPISGHNSLFWYRQTMMRGLELLIYFNNNVPIDDSGMPEDRFSAKMPNASFSTLKIQPSEPRDSAVYFCASSTVGGEDYGYTFGSGTRLTVVE

SEQ ID NO: 71 - protein, 311 aa, Artificial Sequence
  TCR amino acid sequence, Donor HD4
MDSWTFCCVSLCILVAKHTDAGVIQSPRHEVTEMGQEVTLRCKPISGHNSLFWYRQTMMRGLELLIYFNNNVPIDDSGMPEDRFSAKMPNASFSTLKIQPSEPRDSAVYFCASSTVGGEDYGYTFGSGTRLTVVEDLNKVFPPEVAVFEPSEAEISHTQKATLVCLATGFFPDHVELSWWVNGKEVHSGVSTDPQPLKEQPALNDSRYCLSSRLRVSATFWQNPRNHFRCQVQFYGLSENDEWTQDRAKPVTQIVSAEAWGRADCGFTSVSYQQGVLSATILYEILLGKATLYAVLVSALVLMAMVKRKDF

SEQ ID NO: 72 - protein, 313 aa, Artificial Sequence
  TCR amino acid sequence, Donor HD4
MDSWTFCCVSLCILVAKHTDAGVIQSPRHEVTEMGQEVTLRCKPISGHNSLFWYRQTMMRGLELLIYFNNNVPIDDSGMPEDRFSAKMPNASFSTLKIQPSEPRDSAVYFCASSTVGGEDYGYTFGSGTRLTVVEDLKNVFPPEVAVFEPSEAEISHTQKATLVCLATGFYPDHVELSWWVNGKEVHSGVSTDPQPLKEQPALNDSRYCLSSRLRVSATFWQNPRNHFRCQVQFYGLSENDEWTQDRAKPVTQIVSAEAWGRADCGFTSESYQQGVLSATILYEILLGKATLYAVLVSALVLMAMVKRKDSRG

SEQ ID NO: 73 - protein, 6 aa, Artificial Sequence
  TCR amino acid sequence, Donor HD5
DSASNY

SEQ ID NO: 74 - protein, 7 aa, Artificial Sequence
  TCR amino acid sequence, Donor HD5
IRSNVGE

SEQ ID NO: 75 - protein, 15 aa, Artificial Sequence
  TCR amino acid sequence, Donor HD5
CAASMAGAGSYQLTF

SEQ ID NO: 76 - protein, 134 aa, Artificial Sequence
  TCR amino acid sequence, Donor HD5
MTSIRAVFIFLWLQLDLVNGENVEQHPSTLSVQEGDSAVIKCTYSDSASNYFPWYKQELGKRPQLIIDIRSNVGEKKDQRIAVTLNKTAKHFSLHITETQPEDSAVYFCAASMAGAGSYQLTFGKGTKLSVIPN

SEQ ID NO: 77 - protein, 274 aa, Artificial Sequence
  TCR amino acid sequence, Donor HD5
MTSIRAVFIFLWLQLDLVNGENVEQHPSTLSVQEGDSAVIKCTYSDSASNYFPWYKQELGKRPQLIIDIRSNVGEKKDQRIAVTLNKTAKHFSLHITETQPEDSAVYFCAASMAGAGSYQLTFGKGTKLSVIPNIQNPDPAVYQLRDSKSSDKSVCLFTDFDSQTNVSQSKDSDVYITDKTVLDMRSMDFKSNSAVAWSNKSDFACANAFNNSIIPEDTFFPSPESSCDVKLVEKSFETDTNLNFQNLSVIGFRILLLKVAGFNLLMTLRLWSS

SEQ ID NO: 78 - protein, 5 aa, Artificial Sequence
  TCR amino acid sequence, Donor HD5
ENHRY

SEQ ID NO: 79 - protein, 6 aa, Artificial Sequence
  TCR amino acid sequence, Donor HD5
SYGVKD

SEQ ID NO: 80 - protein, 15 aa, Artificial Sequence
  TCR amino acid sequence, Donor HD5
CAISVGQGALYEQYF

SEQ ID NO: 81 - protein, 134 aa, Artificial Sequence
  TCR amino acid sequence, Donor HD5
MGTRLFFYVALCLLWTGHMDAGITQSPRHKVTETGTPVTLRCHQTENHRYMYWYRQDPGHGLRLIHYSYGVKDTDKGEVSDGYSVSRSKTEDFLLTLESATSSQTSVYFCAISVGQGALYEQYFGPGTRLTVTE

SEQ ID NO: 82 - protein, 310 aa, Artificial Sequence
  TCR amino acid sequence, Donor HD5
MGTRLFFYVALCLLWTGHMDAGITQSPRHKVTETGTPVTLRCHQTENHRYMYWYRQDPGHGLRLIHYSYGVKDTDKGEVSDGYSVSRSKTEDFLLTLESATSSQTSVYFCAISVGQGALYEQYFGPGTRLTVTEDLNKVFPPEVAVFEPSEAEISHTQKATLVCLATGFFPDHVELSWWVNGKEVHSGVSTDPQPLKEQPALNDSRYCLSSRLRVSATFWQNPRNHFRCQVQFYGLSENDEWTQDRAKPVTQIVSAEAWGRADCGFTSVSYQQGVLSATILYEILLGKATLYAVLVSALVLMAMVKRKDF

SEQ ID NO: 83 - protein, 312 aa, Artificial Sequence
  TCR amino acid sequence, Donor HD5
MGTRLFFYVALCLLWTGHMDAGITQSPRHKVTETGTPVTLRCHQTENHRYMYWYRQDPGHGLRLIHYSYGVKDTDKGEVSDGYSVSRSKTEDFLLTLESATSSQTSVYFCAISVGQGALYEQYFGPGTRLTVTEDLKNVFPPEVAVFEPSEAEISHTQKATLVCLATGFYPDHVELSWWVNGKEVHSGVSTDPQPLKEQPALNDSRYCLSSRLRVSATFWQNPRNHFRCQVQFYGLSENDEWTQDRAKPVTQIVSAEAWGRADCGFTSESYQQGVLSATILYEILLGKATLYAVLVSALVLMAMVKRKDSRG

SEQ ID NO: 84 - protein, 5 aa, Artificial Sequence
  TCR amino acid sequence, Donor HD5
SGDLS

SEQ ID NO: 85 - protein, 6 aa, Artificial Sequence
  TCR amino acid sequence, Donor HD5
YYNGEE

SEQ ID NO: 86 - protein, 16 aa, Artificial Sequence
  TCR amino acid sequence, Donor HD5
CASSVARDRRNYGYTF

SEQ ID NO: 87 - protein, 135 aa, Artificial Sequence
  TCR amino acid sequence, Donor HD5
MGFRLLCCVAFCLLGAGPVDSGVTQTPKHLITATGQRVTLRCSPRSGDLSVYWYQQSLDQGLQFLIQYYNGEERAKGNILERFSAQQFPDLHSELNLSSLELGDSALYFCASSVARDRRNYGYTFGSGTRLTVVE

SEQ ID NO: 88 - protein, 311 aa, Artificial Sequence
  TCR amino acid sequence, Donor HD5
MGFRLLCCVAFCLLGAGPVDSGVTQTPKHLITATGQRVTLRCSPRSGDLSVYWYQQSLDQGLQFLIQYYNGEERAKGNILERFSAQQFPDLHSELNLSSLELGDSALYFCASSVARDRRNYGYTFGSGTRLTVVEDLNKVFPPEVAVFEPSEAEISHTQKATLVCLATGFFPDHVELSWWVNGKEVHSGVSTDPQPLKEQPALNDSRYCLSSRLRVSATFWQNPRNHFRCQVQFYGLSENDEWTQDRAKPVTQIVSAEAWGRADCGFTSVSYQQGVLSATILYEILLGKATLYAVLVSALVLMAMVKRKDF

SEQ ID NO: 89 - protein, 313 aa, Artificial Sequence
  TCR amino acid sequence, Donor HD5
MGFRLLCCVAFCLLGAGPVDSGVTQTPKHLITATGQRVTLRCSPRSGDLSVYWYQQSLDQGLQFLIQYYNGEERAKGNILERFSAQQFPDLHSELNLSSLELGDSALYFCASSVARDRRNYGYTFGSGTRLTVVEDLKNVFPPEVAVFEPSEAEISHTQKATLVCLATGFYPDHVELSWWVNGKEVHSGVSTDPQPLKEQPALNDSRYCLSSRLRVSATFWQNPRNHFRCQVQFYGLSENDEWTQDRAKPVTQIVSAEAWGRADCGFTSESYQQGVLSATILYEILLGKATLYAVLVSALVLMAMVKRKDSRG

SEQ ID NO: 90 - protein, 6 aa, Artificial Sequence
  TCR amino acid sequence, Donor HD6
NSMFDY

SEQ ID NO: 91 - protein, 7 aa, Artificial Sequence
  TCR amino acid sequence, Donor HD6
ISSIKDK

SEQ ID NO: 92 - protein, 10 aa, Artificial Sequence
  TCR amino acid sequence, Donor HD6
CAANNARLMF

SEQ ID NO: 93 - protein, 136 aa, Artificial Sequence
  TCR amino acid sequence, Donor HD6
MAMLLGASVLILWLQPDWVNSQQKNDDQQVKQNSPSLSVQEGRISILNCDYTNSMFDYFLWYKKYPAEGPTFLISISSIKDKNEDGRFTVFLNKSAKHLSLHIVPSQPGDSAVYFCAANNARLMFGDGTQLVVKPN

SEQ ID NO: 94 - protein, 276 aa, Artificial Sequence
  TCR amino acid sequence, Donor HD6
MAMLLGASVLILWLQPDWVNSQQKNDDQQVKQNSPSLSVQEGRISILNCDYTNSMFDYFLWYKKYPAEGPTFLISISSIKDKNEDGRFTVFLNKSAKHLSLHIVPSQPGDSAVYFCAANNARLMFGDGTQLVVKPNIQNPDPAVYQLRDSKSSDKSVCLFTDFDSQTNVSQSKDSDVYITDKTVLDMRSMDFKSNSAVAWSNKSDFACANAFNNSIIPEDTFFPSPESSCDVKLVEKSFETDTNLNFQNLSVIGFRILLLKVAGFNLLMTLRLWSS

SEQ ID NO: 95 - protein, 5 aa, Artificial Sequence
  TCR amino acid sequence, Donor HD6
SGHNS

SEQ ID NO: 96 - protein, 6 aa, Artificial Sequence
  TCR amino acid sequence, Donor HD6
FNNNVP

SEQ ID NO: 97 - protein, 13 aa, Artificial Sequence
  TCR amino acid sequence, Donor HD6
CASSDTRAREQFF

SEQ ID NO: 98 - protein, 133 aa, Artificial Sequence
  TCR amino acid sequence, Donor HD6
MDSWTFCCVSLCILVAKHTDAGVIQSPRHEVTEMGQEVTLRCKPISGHNSLFWYRQTMMRGLELLIYFNNNVPIDDSGMPEDRFSAKMPNASFSTLKIQPSEPRDSAVYFCASSDTRAREQFFGPGTRLTVLE

SEQ ID NO: 99 - protein, 309 aa, Artificial Sequence
  TCR amino acid sequence, Donor HD6
MDSWTFCCVSLCILVAKHTDAGVIQSPRHEVTEMGQEVTLRCKPISGHNSLFWYRQTMMRGLELLIYFNNNVPIDDSGMPEDRFSAKMPNASFSTLKIQPSEPRDSAVYFCASSDTRAREQFFGPGTRLTVLEDLNKVFPPEVAVFEPSEAEISHTQKATLVCLATGFFPDHVELSWWVNGKEVHSGVSTDPQPLKEQPALNDSRYCLSSRLRVSATFWQNPRNHFRCQVQFYGLSENDEWTQDRAKPVTQIVSAEAWGRADCGFTSVSYQQGVLSATILYEILLGKATLYAVLVSALVLMAMVKRKDF

SEQ ID NO: 100 - protein, 311 aa, Artificial Sequence
  TCR amino acid sequence, Donor HD6
MDSWTFCCVSLCILVAKHTDAGVIQSPRHEVTEMGQEVTLRCKPISGHNSLFWYRQTMMRGLELLIYFNNNVPIDDSGMPEDRFSAKMPNASFSTLKIQPSEPRDSAVYFCASSDTRAREQFFGPGTRLTVLEDLKNVFPPEVAVFEPSEAEISHTQKATLVCLATGFYPDHVELSWWVNGKEVHSGVSTDPQPLKEQPALNDSRYCLSSRLRVSATFWQNPRNHFRCQVQFYGLSENDEWTQDRAKPVTQIVSAEAWGRADCGFTSESYQQGVLSATILYEILLGKATLYAVLVSALVLMAMVKRKDSRG

SEQ ID NO: 101 - protein, 6 aa, Artificial Sequence
  TCR amino acid sequence, Donor HD7
DSSSTY

SEQ ID NO: 102 - protein, 7 aa, Artificial Sequence
  TCR amino acid sequence, Donor HD7
IFSNMDM

SEQ ID NO: 103 - protein, 12 aa, Artificial Sequence
  TCR amino acid sequence, Donor HD7
CAERLNTDKLIF

SEQ ID NO: 104 - protein, 132 aa, Artificial Sequence
  TCR amino acid sequence, Donor HD7
MKTFAGFSFLFLWLQLDCMSRGEDVEQSLFLSVREGDSSVINCTYTDSSSTYLYWYKQEPGAGLQLLTYIFSNMDMKQDQRLTVLLNKKDKHLSLRIADTQTGDSAIYFCAERLNTDKLIFGTGTRLQVFPN

SEQ ID NO: 105 - protein, 272 aa, Artificial Sequence
  TCR amino acid sequence, Donor HD7
MKTFAGFSFLFLWLQLDCMSRGEDVEQSLFLSVREGDSSVINCTYTDSSSTYLYWYKQEPGAGLQLLTYIFSNMDMKQDQRLTVLLNKKDKHLSLRIADTQTGDSAIYFCAERLNTDKLIFGTGTRLQVFPNIQNPDPAVYQLRDSKSSDKSVCLFTDFDSQTNVSQSKDSDVYITDKTVLDMRSMDFKSNSAVAWSNKSDFACANAFNNSIIPEDTFFPSPESSCDVKLVEKSFETDTNLNFQNLSVIGFRILLLKVAGFNLLMTLRLWSS

SEQ ID NO: 106 - protein, 5 aa, Artificial Sequence
  TCR amino acid sequence, Donor HD7
DSVNN

SEQ ID NO: 107 - protein, 5 aa, Artificial Sequence
  TCR amino acid sequence, Donor HD7
IPSGT

SEQ ID NO: 108 - protein, 14 aa, Artificial Sequence
  TCR amino acid sequence, Donor HD7
CAVEATDSWGKLQF

SEQ ID NO: 109 - protein, 131 aa, Artificial Sequence
  TCR amino acid sequence, Donor HD7
MKRILGALLGLLSAQVCCVRGIQVEQSPPDLILQEGANSTLRCNFSDSVNNLQWFHQNPWGQLINLFYIPSGTKQNGRLSATTVATERYSLLYISSSQTTDSGVYFCAVEATDSWGKLQFGAGTQVVVTPD

SEQ ID NO: 110 - protein, 271 aa, Artificial Sequence
  TCR amino acid sequence, Donor HD7
MKRILGALLGLLSAQVCCVRGIQVEQSPPDLILQEGANSTLRCNFSDSVNNLQWFHQNPWGQLINLFYIPSGTKQNGRLSATTVATERYSLLYISSSQTTDSGVYFCAVEATDSWGKLQFGAGTQVVVTPDIQNPDPAVYQLRDSKSSDKSVCLFTDFDSQTNVSQSKDSDVYITDKTVLDMRSMDFKSNSAVAWSNKSDFACANAFNNSIIPEDTFFPSPESSCDVKLVEKSFETDTNLNFQNLSVIGFRILLLKVAGFNLLMTLRLWSS

SEQ ID NO: 111 - protein, 6 aa, Artificial Sequence
  TCR amino acid sequence, Donor HD7
DSASNY

SEQ ID NO: 112 - protein, 7 aa, Artificial Sequence
  TCR amino acid sequence, Donor HD7
IRSNVGE

SEQ ID NO: 113 - protein, 12 aa, Artificial Sequence
  TCR amino acid sequence, Donor HD7
CAVRTSYDKVIF

SEQ ID NO: 114 - protein, 131 aa, Artificial Sequence
  TCR amino acid sequence, Donor HD7
MTSIRAVFIFLWLQLDLVNGENVEQHPSTLSVQEGDSAVIKCTYSDSASNYFPWYKQELGKRPQLIIDIRSNVGEKKDQRIAVTLNKTAKHFSLHITETQPEDSAVYFCAVRTSYDKVIFGPGTSLSVIPN

SEQ ID NO: 115 - protein, 15 aa, Artificial Sequence
  Wilms tumour 1 (WT1) peptide 40
AAQWAPVLDFAPPGA

SEQ ID NO: 116 - protein, 15 aa, Artificial Sequence
  WT1 peptide 41
APVLDFAPPGASAYG

SEQ ID NO: 117 - protein, 11 aa, Artificial Sequence
  WT1 peptide Overlapping sequence
APVLDFAPPGA

SEQ ID NO: 118 - protein, 15 aa, Artificial Sequence
  WT1 peptide 54
QCLSAFTVHFSGQFT

SEQ ID NO: 119 - protein, 15 aa, Artificial Sequence
  WT1 peptide 77
EDPMGQQGSLGEQQY

SEQ ID NO: 120 - protein, 15 aa, Artificial Sequence
  WT1 peptide 90
SQLECMTWNQMNLGA

SEQ ID NO: 121 - protein, 15 aa, Artificial Sequence
  WT1 peptide 17
TCVPEPASQHTLRSG

SEQ ID NO: 122 - protein, 15 aa, Artificial Sequence
  WT1 peptide 18
EPASQHTLRSGPGCL

SEQ ID NO: 123 - protein, 11 aa, Artificial Sequence
  WT1 peptide Overlapping sequence
EPASQHTLRSG

SEQ ID NO: 124 - protein, 15 aa, Artificial Sequence
  WT1 peptide 99
HSTGYESDNHTTPIL

SEQ ID NO: 125 - protein, 15 aa, Artificial Sequence
  WT1 peptide 100
YESDNHTTPILCGAQ

SEQ ID NO: 126 - protein, 11 aa, Artificial Sequence
  WT1 peptide Overlapping sequence
YESDNHTTPIL

SEQ ID NO: 127 - protein, 15 aa, Artificial Sequence
  WT1 peptide 101
NHTTPILCGAQYRIH

SEQ ID NO: 128 - protein, 140 aa, Artificial Sequence
  sequence of an alpha chain constant domain encoded by a TRAC gene
IQNPDPAVYQLRDSKSSDKSVCLFTDFDSQTNVSQSKDSDVYITDKTVLDMRSMDFKSNSAVAWSNKSDFACANAFNNSIIPEDTFFPSPESSCDVKLVEKSFETDTNLNFQNLSVIGFRILLLKVAGFNLLMTLRLWSS

SEQ ID NO: 129 - protein, 176 aa, Artificial Sequence
  sequence of a beta chain constant domain encoded by a TRBC1 gene
DLNKVFPPEVAVFEPSEAEISHTQKATLVCLATGFFPDHVELSWWVNGKEVHSGVSTDPQPLKEQPALNDSRYCLSSRLRVSATFWQNPRNHFRCQVQFYGLSENDEWTQDRAKPVTQIVSAEAWGRADCGFTSVSYQQGVLSATILYEILLGKATLYAVLVSALVLMAMVKRKDF

SEQ ID NO: 130 - protein, 178 aa, Artificial Sequence
  sequence of a beta chain constant domain encoded by a TRBC2 gene
DLKNVFPPEVAVFEPSEAEISHTQKATLVCLATGFYPDHVELSWWVNGKEVHSGVSTDPQPLKEQPALNDSRYCLSSRLRVSATFWQNPRNHFRCQVQFYGLSENDEWTQDRAKPVTQIVSAEAWGRADCGFTSESYQQGVLSATILYEILLGKATLYAVLVSALVLMAMVKRKDSRG

SEQ ID NO: 131 - protein, 575 aa, Artificial Sequence
  WT1 protein sequence
SRQRPHPGALRNPTACPLPHFPPSLPPTHSPTHPPRAGTAAQAPGPRRLLAAILDFLLLQDPASTCVPEPASQHTLRSGPGCLQQPEQQGVRDPGGIWAKLGAAEASAERLQGRRSRGASGSEPQQMGSDVRDLNALLPAVPSLGGGGGCALPVSGAAQWAPVLDFAPPGASAYGSLGGPAPPPAPPPPPPPPPHSFIKQEPSWGGAEPHEEQCLSAFTVHFSGQFTGTAGACRYGPFGPPPPSQASSGQARMFPNAPYLPSCLESQPAIRNQGYSTVTFDGTPSYGHTPSHHAAQFPNHSFKHEDPMGQQGSLGEQQYSVPPPVYGCHTPTDSCTGSQALLLRTPYSSDNLYQMTSQLECMTWNQMNLGATLKGVAAGSSSSVKWTEGQSNHSTGYESDNHTTPILCGAQYRIHTHGVFRGIQDVRRVPGVAPTLVRSASETSEKRPFMCAYPGCNKRYFKLSHLQMHSRKHTGEKPYQCDFKDCERRFSRSDQLKRHQRRHTGVKPFQCKTCQRKFSRSDHLKTHTRTHTGKTSEKPFSCRWPSCQKKFARSDELVRHHNMHQRNMTKLQLAL

SEQ ID NO: 132 - DNA, 816 bp, Artificial Sequence
  Nucleotide sequence encoding TCR, Donor HD1
atggagactctcctgaaagtgctttcaggcaccttgttgtggcagttgacctgggtgagaagccaacaaccagtgcagagtcctcaagccgtgatcctccgagaaggggaagatgctgtcatcaactgcagttcctccaaggctttatattctgtacactggtacaggcagaagcatggtgaagcacccgtcttcctgatgatattactgaagggtggagaacagaagggtcatgaaaaaatatctgcttcatttaatgaaaaaaagcagcaaagctccctgtaccttacggcctcccagctcagttactcaggaacctacttctgcggcacagcttggattaacgactacaagctcagctttggagccggaaccacagtaactgtaagagcaaatatccagaaccctgaccctgccgtgtaccagctgagagactctaaatccagtgacaagtctgtctgcctattcaccgattttgattctcaaacaaatgtgtcacaaagtaaggattctgatgtgtatatcacagacaaaactgtgctagacatgaggtctatggacttcaagagcaacagtgctgtggcctggagcaacaaatctgactttgcatgtgcaaacgccttcaacaacagcattattccagaagacaccttcttccccagcccagaaagttcctgtgatgtcaagctggtcgagaaaagctttgaaacagatacgaacctaaactttcaaaacctgtcagtgattgggttccgaatcctcctcctgaaagtggccgggtttaatctgctcatgacgctgcggctgtggtccagc

SEQ ID NO: 133 - DNA, 936 bp, Artificial Sequence
  Nucleotide sequence encoding TCR, Donor HD1
atgggctcctggaccctctgctgtgtgtccctttgcatcctggtagcaaagcacacagatgctggagttatccagtcaccccggcacgaggtgacagagatgggacaagaagtgactctgagatgtaaaccaatttcaggacacgactaccttttctggtacagacagaccatgatgcggggactggagttgctcatttactttaacaacaacgttccgatagatgattcagggatgcccgaggatcgattctcagctaagatgcctaatgcatcattctccactctgaagatccagccctcagaacccagggactcagctgtgtacttctgtgccagcagaaaaaccgggggatatagcaatcagccccagcattttggtgatgggactcgactctccatcctagaggacctgaacaaggtgttcccacccgaggtcgctgtgtttgagccatcagaagcagagatctcccacacccaaaaggccacactggtgtgcctggccacaggcttcttccccgaccacgtggagctgagctggtgggtgaatgggaaggaggtgcacagtggggtcagcacggacccgcagcccctcaaggagcagcccgccctcaatgactccagatactgcctgagcagccgcctgagggtctcggccaccttctggcagaacccccgcaaccacttccgctgtcaagtccagttctacgggctctcggagaatgacgagtggacccaggatagggccaaacccgtcacccagatcgtcagcgccgaggcctggggtagagcagactgtggctttacctcggtgtcctaccagcaaggggtcctgtctgccaccatcctctatgagatcctgctagggaaggccaccctgtatgctgtgctggtcagcgcccttgtgttgatggccatggtcaagagaaaggatttc

SEQ ID NO: 134 - DNA, 942 bp, Artificial Sequence
  Nucleotide sequence encoding TCR, Donor HD1
atgggctcctggaccctctgctgtgtgtccctttgcatcctggtagcaaagcacacagatgctggagttatccagtcaccccggcacgaggtgacagagatgggacaagaagtgactctgagatgtaaaccaatttcaggacacgactaccttttctggtacagacagaccatgatgcggggactggagttgctcatttactttaacaacaacgttccgatagatgattcagggatgcccgaggatcgattctcagctaagatgcctaatgcatcattctccactctgaagatccagccctcagaacccagggactcagctgtgtacttctgtgccagcagaaaaaccgggggatatagcaatcagccccagcattttggtgatgggactcgactctccatcctagaggacctgaaaaacgtgttcccacccgaggtcgctgtgtttgagccatcagaagcagagatctcccacacccaaaaggccacactggtgtgcctggccacaggcttctaccccgaccacgtggagctgagctggtgggtgaatgggaaggaggtgcacagtggggtcagcacagacccgcagcccctcaaggagcagcccgccctcaatgactccagatactgcctgagcagccgcctgagggtctcggccaccttctggcagaacccccgcaaccacttccgctgtcaagtccagttctacgggctctcggagaatgacgagtggacccaggatagggccaaacctgtcacccagatcgtcagcgccgaggcctggggtagagcagactgtggcttcacctccgagtcttaccagcaaggggtcctgtctgccaccatcctctatgagatcttgctagggaaggccaccttgtatgccgtgctggtcagtgccctcgtgctgatggccatggtcaagagaaaggattccagaggc

SEQ ID NO: 135 - DNA, 822 bp, Artificial Sequence
  Nucleotide sequence encoding TCR, Donor HD2-1
atgctcctgctgctcgtcccagtgctcgaggtgatttttaccctgggaggaaccagagcccagtcggtgacccagcttggcagccacgtctctgtctctgaaggagccctggttctgctgaggtgcaactactcatcgtctgttccaccatatctcttctggtatgtgcaataccccaaccaaggactccagcttctcctgaagtacacatcagcggccaccctggttaaaggcatcaacggttttgaggctgaatttaagaagagtgaaacctccttccacctgacgaaaccctcagcccatatgagcgacgcggctgagtacttctgtgctgtgagattatctggttctgcaaggcaactgacctttggatctgggacacaattgactgttttacctgatatccagaaccctgaccctgccgtgtaccagctgagagactctaaatccagtgacaagtctgtctgcctattcaccgattttgattctcaaacaaatgtgtcacaaagtaaggattctgatgtgtatatcacagacaaaactgtgctagacatgaggtctatggacttcaagagcaacagtgctgtggcctggagcaacaaatctgactttgcatgtgcaaacgccttcaacaacagcattattccagaagacaccttcttccccagcccagaaagttcctgtgatgtcaagctggtcgagaaaagctttgaaacagatacgaacctaaactttcaaaacctgtcagtgattgggttccgaatcctcctcctgaaagtggccgggtttaatctgctcatgacgctgcggctgtggtccagc

SEQ ID NO: 136 - DNA, 924 bp, Artificial Sequence
  Nucleotide sequence encoding TCR, Donor HD2-1
atgggcaccaggctcctctgctgggcggccctctgtctcctgggagcagaactcacagaagctggagttgcccagtctcccagatataagattatagagaaaaggcagagtgtggctttttggtgcaatcctatatctggccatgctaccctttactggtaccagcagatcctgggacagggcccaaagcttctgattcagtttcagaataacggtgtagtggatgattcacagttgcctaaggatcgattttctgcagagaggctcaaaggagtagactccactctcaagatccagcctgcaaagcttgaggactcggccgtgtatctctgtgccagcagcttactgggagacgagcagtacttcgggccgggcaccaggctcacggtcacagaggacctgaacaaggtgttcccacccgaggtcgctgtgtttgagccatcagaagcagagatctcccacacccaaaaggccacactggtgtgcctggccacaggcttcttccccgaccacgtggagctgagctggtgggtgaatgggaaggaggtgcacagtggggtcagcacggacccgcagcccctcaaggagcagcccgccctcaatgactccagatactgcctgagcagccgcctgagggtctcggccaccttctggcagaacccccgcaaccacttccgctgtcaagtccagttctacgggctctcggagaatgacgagtggacccaggatagggccaaacccgtcacccagatcgtcagcgccgaggcctggggtagagcagactgtggctttacctcggtgtcctaccagcaaggggtcctgtctgccaccatcctctatgagatcctgctagggaaggccaccctgtatgctgtgctggtcagcgcccttgtgttgatggccatggtcaagagaaaggatttc

SEQ ID NO: 137 - DNA, 930 bp, Artificial Sequence
  Nucleotide sequence encoding TCR, Donor HD2-1
atgggcaccaggctcctctgctgggcggccctctgtctcctgggagcagaactcacagaagctggagttgcccagtctcccagatataagattatagagaaaaggcagagtgtggctttttggtgcaatcctatatctggccatgctaccctttactggtaccagcagatcctgggacagggcccaaagcttctgattcagtttcagaataacggtgtagtggatgattcacagttgcctaaggatcgattttctgcagagaggctcaaaggagtagactccactctcaagatccagcctgcaaagcttgaggactcggccgtgtatctctgtgccagcagcttactgggagacgagcagtacttcgggccgggcaccaggctcacggtcacagaggacctgaaaaacgtgttcccacccgaggtcgctgtgtttgagccatcagaagcagagatctcccacacccaaaaggccacactggtgtgcctggccacaggcttctaccccgaccacgtggagctgagctggtgggtgaatgggaaggaggtgcacagtggggtcagcacagacccgcagcccctcaaggagcagcccgccctcaatgactccagatactgcctgagcagccgcctgagggtctcggccaccttctggcagaacccccgcaaccacttccgctgtcaagtccagttctacgggctctcggagaatgacgagtggacccaggatagggccaaacctgtcacccagatcgtcagcgccgaggcctggggtagagcagactgtggcttcacctccgagtcttaccagcaaggggtcctgtctgccaccatcctctatgagatcttgctagggaaggccaccttgtatgccgtgctggtcagtgccctcgtgctgatggccatggtcaagagaaaggattccagaggc

SEQ ID NO: 138 - DNA, 828 bp, Artificial Sequence
  Nucleotide sequence encoding TCR, Donor HD2-2
atggcatgccctggcttcctgtgggcacttgtgatctccacctgtcttgaatttagcatggctcagacagtcactcagtctcaaccagagatgtctgtgcaggaggcagagaccgtgaccctgagctgcacatatgacaccagtgagagtgattattatttattctggtacaagcagcctcccagcaggcagatgattctcgttattcgccaagaagcttataagcaacagaatgcaacagagaatcgtttctctgtgaacttccagaaagcagccaaatccttcagtctcaagatctcagactcacagctgggggatgccgcgatgtatttctgtgcttataggagtctaaaatatggaaacaaactggtctttggcgcaggaaccattctgagagtcaagtcctatatccagaaccctgaccctgccgtgtaccagctgagagactctaaatccagtgacaagtctgtctgcctattcaccgattttgattctcaaacaaatgtgtcacaaagtaaggattctgatgtgtatatcacagacaaaactgtgctagacatgaggtctatggacttcaagagcaacagtgctgtggcctggagcaacaaatctgactttgcatgtgcaaacgccttcaacaacagcattattccagaagacaccttcttccccagcccagaaagttcctgtgatgtcaagctggtcgagaaaagctttgaaacagatacgaacctaaactttcaaaacctgtcagtgattgggttccgaatcctcctcctgaaagtggccgggtttaatctgctcatgacgctgcggctgtggtccagc

SEQ ID NO: 139 - DNA, 936 bp, Artificial Sequence
  Nucleotide sequence encoding TCR, Donor HD2-2
atgggcaccaggctcctcttctgggtggccttctgtctcctgggggcagatcacacaggagctggagtctcccagtcccccagtaacaaggtcacagagaagggaaaggatgtagagctcaggtgtgatccaatttcaggtcatactgccctttactggtaccgacagagcctggggcagggcctggagtttttaatttacttccaaggcaacagtgcaccagacaaatcagggctgcccagtgatcgcttctctgcagagaggactgggggatccgtctccactctgacgatccagcgcacacagcaggaggactcggccgtgtatctctgtgccagcagcttggtagctttacagggtgcgggcgagcagtacttcgggccgggcaccaggctcacggtcacagaggacctgaacaaggtgttcccacccgaggtcgctgtgtttgagccatcagaagcagagatctcccacacccaaaaggccacactggtgtgcctggccacaggcttcttccccgaccacgtggagctgagctggtgggtgaatgggaaggaggtgcacagtggggtcagcacggacccgcagcccctcaaggagcagcccgccctcaatgactccagatactgcctgagcagccgcctgagggtctcggccaccttctggcagaacccccgcaaccacttccgctgtcaagtccagttctacgggctctcggagaatgacgagtggacccaggatagggccaaacccgtcacccagatcgtcagcgccgaggcctggggtagagcagactgtggctttacctcggtgtcctaccagcaaggggtcctgtctgccaccatcctctatgagatcctgctagggaaggccaccctgtatgctgtgctggtcagcgcccttgtgttgatggccatggtcaagagaaaggatttc

SEQ ID NO: 140 - DNA, 942 bp, Artificial Sequence
  Nucleotide sequence encoding TCR, Donor HD2-2
atgggcaccaggctcctcttctgggtggccttctgtctcctgggggcagatcacacaggagctggagtctcccagtcccccagtaacaaggtcacagagaagggaaaggatgtagagctcaggtgtgatccaatttcaggtcatactgccctttactggtaccgacagagcctggggcagggcctggagtttttaatttacttccaaggcaacagtgcaccagacaaatcagggctgcccagtgatcgcttctctgcagagaggactgggggatccgtctccactctgacgatccagcgcacacagcaggaggactcggccgtgtatctctgtgccagcagcttggtagctttacagggtgcgggcgagcagtacttcgggccgggcaccaggctcacggtcacagaggacctgaaaaacgtgttcccacccgaggtcgctgtgtttgagccatcagaagcagagatctcccacacccaaaaggccacactggtgtgcctggccacaggcttctaccccgaccacgtggagctgagctggtgggtgaatgggaaggaggtgcacagtggggtcagcacagacccgcagcccctcaaggagcagcccgccctcaatgactccagatactgcctgagcagccgcctgagggtctcggccaccttctggcagaacccccgcaaccacttccgctgtcaagtccagttctacgggctctcggagaatgacgagtggacccaggatagggccaaacctgtcacccagatcgtcagcgccgaggcctggggtagagcagactgtggcttcacctccgagtcttaccagcaaggggtcctgtctgccaccatcctctatgagatcttgctagggaaggccaccttgtatgccgtgctggtcagtgccctcgtgctgatggccatggtcaagagaaaggattccagaggc

SEQ ID NO: 141 - DNA, 822 bp, Artificial Sequence
  Nucleotide sequence encoding TCR, Donor HD3
atgatatccttgagagttttactggtgatcctgtggcttcagttaagctgggtttggagccaacggaaggaggtggagcaggatcctggacccttcaatgttccagagggagccactgtcgctttcaactgtacttacagcaacagtgcttctcagtctttcttctggtacagacaggattgcaggaaagaacctaagttgctgatgtccgtatactccagtggtaatgaagatggaaggtttacagcacagctcaatagagccagccagtatatttccctgctcatcagagactccaagctcagtgattcagccacctacctctgtgtggtgaacctcctgtctaaccagggaggaaagcttatcttcggacagggaacggagttatctgtgaaacccaatatccagaaccctgaccctgccgtgtaccagctgagagactctaaatccagtgacaagtctgtctgcctattcaccgattttgattctcaaacaaatgtgtcacaaagtaaggattctgatgtgtatatcacagacaaaactgtgctagacatgaggtctatggacttcaagagcaacagtgctgtggcctggagcaacaaatctgactttgcatgtgcaaacgccttcaacaacagcattattccagaagacaccttcttccccagcccagaaagttcctgtgatgtcaagctggtcgagaaaagctttgaaacagatacgaacctaaactttcaaaacctgtcagtgattgggttccgaatcctcctcctgaaagtggccgggtttaatctgctcatgacgctgcggctgtggtccagc

SEQ ID NO: 142 - DNA, 942 bp, Artificial Sequence
  Nucleotide sequence encoding TCR, Donor HD3
atgggctgcaggctgctctgctgtgcggttctctgtctcctgggagcgggtgagttggtccccatggaaacgggagttacgcagacaccaagacacctggtcatgggaatgacaaataagaagtctttgaaatgtgaacaacatctgggtcataacgctatgtattggtacaagcaaagtgctaagaagccactggagctcatgtttgtctacagtcttgaagaacgggttgaaaacaacagtgtgccaagtcgcttctcacctgaatgccccaacagctctcacttattccttcacctacacaccctgcagccagaagactcggccctgtatctctgcgccagcagccaagattacttggtttctaatgaaaaactgttttttggcagtggaacccagctctctgtcttggaggacctgaacaaggtgttcccacccgaggtcgctgtgtttgagccatcagaagcagagatctcccacacccaaaaggccacactggtgtgcctggccacaggcttcttccccgaccacgtggagctgagctggtgggtgaatgggaaggaggtgcacagtggggtcagcacggacccgcagcccctcaaggagcagcccgccctcaatgactccagatactgcctgagcagccgcctgagggtctcggccaccttctggcagaacccccgcaaccacttccgctgtcaagtccagttctacgggctctcggagaatgacgagtggacccaggatagggccaaacccgtcacccagatcgtcagcgccgaggcctggggtagagcagactgtggctttacctcggtgtcctaccagcaaggggtcctgtctgccaccatcctctatgagatcctgctagggaaggccaccctgtatgctgtgctggtcagcgcccttgtgttgatggccatggtcaagagaaaggatttc

SEQ ID NO: 143 - DNA, 948 bp, Artificial Sequence
  Nucleotide sequence encoding TCR, Donor HD3
atgggctgcaggctgctctgctgtgcggttctctgtctcctgggagcgggtgagttggtccccatggaaacgggagttacgcagacaccaagacacctggtcatgggaatgacaaataagaagtctttgaaatgtgaacaacatctgggtcataacgctatgtattggtacaagcaaagtgctaagaagccactggagctcatgtttgtctacagtcttgaagaacgggttgaaaacaacagtgtgccaagtcgcttctcacctgaatgccccaacagctctcacttattccttcacctacacaccctgcagccagaagactcggccctgtatctctgcgccagcagccaagattacttggtttctaatgaaaaactgttttttggcagtggaacccagctctctgtcttggaggacctgaaaaacgtgttcccacccgaggtcgctgtgtttgagccatcagaagcagagatctcccacacccaaaaggccacactggtgtgcctggccacaggcttctaccccgaccacgtggagctgagctggtgggtgaatgggaaggaggtgcacagtggggtcagcacagacccgcagcccctcaaggagcagcccgccctcaatgactccagatactgcctgagcagccgcctgagggtctcggccaccttctggcagaacccccgcaaccacttccgctgtcaagtccagttctacgggctctcggagaatgacgagtggacccaggatagggccaaacctgtcacccagatcgtcagcgccgaggcctggggtagagcagactgtggcttcacctccgagtcttaccagcaaggggtcctgtctgccaccatcctctatgagatcttgctagggaaggccaccttgtatgccgtgctggtcagtgccctcgtgctgatggccatggtcaagagaaaggattccagaggc

SEQ ID NO: 144 - DNA, 819 bp, Artificial Sequence
  Nucleotide sequence encoding TCR, Donor HD4-1
atggaaactctcctgggagtgtctttggtgattctatggcttcaactggctagggtgaacagtcaacagggagaagaggatcctcaggccttgagcatccaggagggtgaaaatgccaccatgaactgcagttacaaaactagtataaacaatttacagtggtatagacaaaattcaggtagaggccttgtccacctaattttaatacgttcaaatgaaagagagaaacacagtggaagattaagagtcacgcttgacacttccaagaaaagcagttccttgttgatcacggcttcccgggcagcagacactgcttcttacttctgtgctacggacgcgtattcaggaaacacacctcttgtctttggaaagggcacaagactttctgtgattgcaaatatccagaaccctgaccctgccgtgtaccagctgagagactctaaatccagtgacaagtctgtctgcctattcaccgattttgattctcaaacaaatgtgtcacaaagtaaggattctgatgtgtatatcacagacaaaactgtgctagacatgaggtctatggacttcaagagcaacagtgctgtggcctggagcaacaaatctgactttgcatgtgcaaacgccttcaacaacagcattattccagaagacaccttcttccccagcccagaaagttcctgtgatgtcaagctggtcgagaaaagctttgaaacagatacgaacctaaactttcaaaacctgtcagtgattgggttccgaatcctcctcctgaaagtggccgggtttaatctgctcatgacgctgcggctgtggtccagc

SEQ ID NO: 145 - DNA, 927 bp, Artificial Sequence
  Nucleotide sequence encoding TCR, Donor HD4-1
atgagcatcgggctcctgtgctgtgtggccttttctctcctgtgggcaagtccagtgaatgctggtgtcactcagaccccaaaattccaggtcctgaagacaggacagagcatgacactgcagtgtgcccaggatatgaaccataactccatgtactggtatcgacaagacccaggcatgggactgaggctgatttattactcagcttctgagggtaccactgacaaaggagaagtccccaatggctacaatgtctccagattaaacaaacgggagttctcgctcaggctggagtcggctgctccctcccagacatctgtgtacttctgtgccagcagggcagcagggttggacactgaagctttctttggacaaggcaccagactcacagttgtagaggacctgaacaaggtgttcccacccgaggtcgctgtgtttgagccatcagaagcagagatctcccacacccaaaaggccacactggtgtgcctggccacaggcttcttccccgaccacgtggagctgagctggtgggtgaatgggaaggaggtgcacagtggggtcagcacggacccgcagcccctcaaggagcagcccgccctcaatgactccagatactgcctgagcagccgcctgagggtctcggccaccttctggcagaacccccgcaaccacttccgctgtcaagtccagttctacgggctctcggagaatgacgagtggacccaggatagggccaaacccgtcacccagatcgtcagcgccgaggcctggggtagagcagactgtggctttacctcggtgtcctaccagcaaggggtcctgtctgccaccatcctctatgagatcctgctagggaaggccaccctgtatgctgtgctggtcagcgcccttgtgttgatggccatggtcaagagaaaggatttc

SEQ ID NO: 146 - DNA, 933 bp, Artificial Sequence
  Nucleotide sequence encoding TCR, Donor HD4-1
atgagcatcgggctcctgtgctgtgtggccttttctctcctgtgggcaagtccagtgaatgctggtgtcactcagaccccaaaattccaggtcctgaagacaggacagagcatgacactgcagtgtgcccaggatatgaaccataactccatgtactggtatcgacaagacccaggcatgggactgaggctgatttattactcagcttctgagggtaccactgacaaaggagaagtccccaatggctacaatgtctccagattaaacaaacgggagttctcgctcaggctggagtcggctgctccctcccagacatctgtgtacttctgtgccagcagggcagcagggttggacactgaagctttctttggacaaggcaccagactcacagttgtagaggacctgaaaaacgtgttcccacccgaggtcgctgtgtttgagccatcagaagcagagatctcccacacccaaaaggccacactggtgtgcctggccacaggcttctaccccgaccacgtggagctgagctggtgggtgaatgggaaggaggtgcacagtggggtcagcacagacccgcagcccctcaaggagcagcccgccctcaatgactccagatactgcctgagcagccgcctgagggtctcggccaccttctggcagaacccccgcaaccacttccgctgtcaagtccagttctacgggctctcggagaatgacgagtggacccaggatagggccaaacctgtcacccagatcgtcagcgccgaggcctggggtagagcagactgtggcttcacctccgagtcttaccagcaaggggtcctgtctgccaccatcctctatgagatcttgctagggaaggccaccttgtatgccgtgctggtcagtgccctcgtgctgatggccatggtcaagagaaaggattccagaggc

SEQ ID NO: 147 - DNA, 825 bp, Artificial Sequence
  Nucleotide sequence encoding TCR, Donor HD4-2
atggagaccctcttgggcctgcttatcctttggctgcagctgcaatgggtgagcagcaaacaggaggtgacgcagattcctgcagctctgagtgtcccagaaggagaaaacttggttctcaactgcagtttcactgatagcgctatttacaacctccagtggtttaggcaggaccctgggaaaggtctcacatctctgttgcttattcagtcaagtcagagagagcaaacaagtggaagacttaatgcctcgctggataaatcatcaggacgtagtactttatacattgcagcttctcagcctggtgactcagccacctacctctgtgctgtccgggcagagatttataaccagggaggaaagcttatcttcggacagggaacggagttatctgtgaaacccaatatccagaaccctgaccctgccgtgtaccagctgagagactctaaatccagtgacaagtctgtctgcctattcaccgattttgattctcaaacaaatgtgtcacaaagtaaggattctgatgtgtatatcacagacaaaactgtgctagacatgaggtctatggacttcaagagcaacagtgctgtggcctggagcaacaaatctgactttgcatgtgcaaacgccttcaacaacagcattattccagaagacaccttcttccccagcccagaaagttcctgtgatgtcaagctggtcgagaaaagctttgaaacagatacgaacctaaactttcaaaacctgtcagtgattgggttccgaatcctcctcctgaaagtggccgggtttaatctgctcatgacgctgcggctgtggtccagc

SEQ ID NO: 148 - DNA, 921 bp, Artificial Sequence
  Nucleotide sequence encoding TCR, Donor HD4-2
atgagcatcagcctcctgtgctgtgcagcctttcctctcctgtgggcaggtccagtgaatgctggtgtcactcagaccccaaaattccgcatcctgaagataggacagagcatgacactgcagtgtacccaggatatgaaccataactacatgtactggtatcgacaagacccaggcatggggctgaagctgatttattattcagttggtgctggtatcactgataaaggagaagtcccgaatggctacaacgtctccagatcaaccacagaggatttcccgctcaggctggagttggctgctccctcccagacatctgtgtacttctgtgccagtacccaaactccctacgagcagtacttcgggccgggcaccaggctcacggtcacagaggacctgaacaaggtgttcccacccgaggtcgctgtgtttgagccatcagaagcagagatctcccacacccaaaaggccacactggtgtgcctggccacaggcttcttccccgaccacgtggagctgagctggtgggtgaatgggaaggaggtgcacagtggggtcagcacggacccgcagcccctcaaggagcagcccgccctcaatgactccagatactgcctgagcagccgcctgagggtctcggccaccttctggcagaacccccgcaaccacttccgctgtcaagtccagttctacgggctctcggagaatgacgagtggacccaggatagggccaaacccgtcacccagatcgtcagcgccgaggcctggggtagagcagactgtggctttacctcggtgtcctaccagcaaggggtcctgtctgccaccatcctctatgagatcctgctagggaaggccaccctgtatgctgtgctggtcagcgcccttgtgttgatggccatggtcaagagaaaggatttc

SEQ ID NO: 149 - DNA, 927 bp, Artificial Sequence
  Nucleotide sequence encoding TCR, Donor HD4-2
atgagcatcagcctcctgtgctgtgcagcctttcctctcctgtgggcaggtccagtgaatgctggtgtcactcagaccccaaaattccgcatcctgaagataggacagagcatgacactgcagtgtacccaggatatgaaccataactacatgtactggtatcgacaagacccaggcatggggctgaagctgatttattattcagttggtgctggtatcactgataaaggagaagtcccgaatggctacaacgtctccagatcaaccacagaggatttcccgctcaggctggagttggctgctccctcccagacatctgtgtacttctgtgccagtacccaaactccctacgagcagtacttcgggccgggcaccaggctcacggtcacagaggacctgaaaaacgtgttcccacccgaggtcgctgtgtttgagccatcagaagcagagatctcccacacccaaaaggccacactggtgtgcctggccacaggcttctaccccgaccacgtggagctgagctggtgggtgaatgggaaggaggtgcacagtggggtcagcacagacccgcagcccctcaaggagcagcccgccctcaatgactccagatactgcctgagcagccgcctgagggtctcggccaccttctggcagaacccccgcaaccacttccgctgtcaagtccagttctacgggctctcggagaatgacgagtggacccaggatagggccaaacctgtcacccagatcgtcagcgccgaggcctggggtagagcagactgtggcttcacctccgagtcttaccagcaaggggtcctgtctgccaccatcctctatgagatcttgctagggaaggccaccttgtatgccgtgctggtcagtgccctcgtgctgatggccatggtcaagagaaaggattccagaggc

SEQ ID NO: 150 - DNA, 933 bp, Artificial Sequence
  Nucleotide sequence encoding TCR, Donor HD4-2
atggactcctggaccttctgctgtgtgtccctttgcatcctggtagcgaagcatacagatgctggagttatccagtcaccccgccatgaggtgacagagatgggacaagaagtgactctgagatgtaaaccaatttcaggccacaactcccttttctggtacagacagaccatgatgcggggactggagttgctcatttactttaacaacaacgttccgatagatgattcagggatgcccgaggatcgattctcagctaagatgcctaatgcatcattctccactctgaagatccagccctcagaacccagggactcagctgtgtacttctgtgccagcagcacagtgggaggggaggattatggctacaccttcggttcggggaccaggttaaccgttgtagaggacctgaacaaggtgttcccacccgaggtcgctgtgtttgagccatcagaagcagagatctcccacacccaaaaggccacactggtgtgcctggccacaggcttcttccccgaccacgtggagctgagctggtgggtgaatgggaaggaggtgcacagtggggtcagcacggacccgcagcccctcaaggagcagcccgccctcaatgactccagatactgcctgagcagccgcctgagggtctcggccaccttctggcagaacccccgcaaccacttccgctgtcaagtccagttctacgggctctcggagaatgacgagtggacccaggatagggccaaacccgtcacccagatcgtcagcgccgaggcctggggtagagcagactgtggctttacctcggtgtcctaccagcaaggggtcctgtctgccaccatcctctatgagatcctgctagggaaggccaccctgtatgctgtgctggtcagcgcccttgtgttgatggccatggtcaagagaaaggatttc

SEQ ID NO: 151 - DNA, 939 bp, Artificial Sequence
  Nucleotide sequence encoding TCR, Donor HD4-2
atggactcctggaccttctgctgtgtgtccctttgcatcctggtagcgaagcatacagatgctggagttatccagtcaccccgccatgaggtgacagagatgggacaagaagtgactctgagatgtaaaccaatttcaggccacaactcccttttctggtacagacagaccatgatgcggggactggagttgctcatttactttaacaacaacgttccgatagatgattcagggatgcccgaggatcgattctcagctaagatgcctaatgcatcattctccactctgaagatccagccctcagaacccagggactcagctgtgtacttctgtgccagcagcacagtgggaggggaggattatggctacaccttcggttcggggaccaggttaaccgttgtagaggacctgaaaaacgtgttcccacccgaggtcgctgtgtttgagccatcagaagcagagatctcccacacccaaaaggccacactggtgtgcctggccacaggcttctaccccgaccacgtggagctgagctggtgggtgaatgggaaggaggtgcacagtggggtcagcacagacccgcagcccctcaaggagcagcccgccctcaatgactccagatactgcctgagcagccgcctgagggtctcggccaccttctggcagaacccccgcaaccacttccgctgtcaagtccagttctacgggctctcggagaatgacgagtggacccaggatagggccaaacctgtcacccagatcgtcagcgccgaggcctggggtagagcagactgtggcttcacctccgagtcttaccagcaaggggtcctgtctgccaccatcctctatgagatcttgctagggaaggccaccttgtatgccgtgctggtcagtgccctcgtgctgatggccatggtcaagagaaaggattccagaggc

SEQ ID NO: 152 - DNA, 822 bp, Artificial Sequence
  Nucleotide sequence encoding TCR, Donor HD5
atgacatccattcgagctgtatttatattcctgtggctgcagctggacttggtgaatggagagaatgtggagcagcatccttcaaccctgagtgtccaggagggagacagcgctgttatcaagtgtacttattcagacagtgcctcaaactacttcccttggtataagcaagaacttggaaaaagacctcagcttattatagacattcgttcaaatgtgggcgaaaagaaagaccaacgaattgctgttacattgaacaagacagccaaacatttctccctgcacatcacagagacccaacctgaagactcggctgtctacttctgtgcagcaagtatggctggggctgggagttaccaactcactttcgggaaggggaccaaactctcggtcataccaaatatccagaaccctgaccctgccgtgtaccagctgagagactctaaatccagtgacaagtctgtctgcctattcaccgattttgattctcaaacaaatgtgtcacaaagtaaggattctgatgtgtatatcacagacaaaactgtgctagacatgaggtctatggacttcaagagcaacagtgctgtggcctggagcaacaaatctgactttgcatgtgcaaacgccttcaacaacagcattattccagaagacaccttcttccccagcccagaaagttcctgtgatgtcaagctggtcgagaaaagctttgaaacagatacgaacctaaactttcaaaacctgtcagtgattgggttccgaatcctcctcctgaaagtggccgggtttaatctgctcatgacgctgcggctgtggtccagc

SEQ ID NO: 153 - DNA, 930 bp, Artificial Sequence
  Nucleotide sequence encoding TCR, Donor HD5
atgggcacaaggttgttcttctatgtggccctttgtctcctgtggacaggacacatggatgctggaatcacccagagcccaagacacaaggtcacagagacaggaacaccagtgactctgagatgtcaccagactgagaaccaccgctatatgtactggtatcgacaagacccggggcatgggctgaggctgatccattactcatatggtgttaaagatactgacaaaggagaagtctcagatggctatagtgtctctagatcaaagacagaggatttcctcctcactctggagtccgctaccagctcccagacatctgtgtacttctgtgccatctcggtgggacagggggccctctacgagcagtacttcgggccgggcaccaggctcacggtcacagaggacctgaacaaggtgttcccacccgaggtcgctgtgtttgagccatcagaagcagagatctcccacacccaaaaggccacactggtgtgcctggccacaggcttcttccccgaccacgtggagctgagctggtgggtgaatgggaaggaggtgcacagtggggtcagcacggacccgcagcccctcaaggagcagcccgccctcaatgactccagatactgcctgagcagccgcctgagggtctcggccaccttctggcagaacccccgcaaccacttccgctgtcaagtccagttctacgggctctcggagaatgacgagtggacccaggatagggccaaacccgtcacccagatcgtcagcgccgaggcctggggtagagcagactgtggctttacctcggtgtcctaccagcaaggggtcctgtctgccaccatcctctatgagatcctgctagggaaggccaccctgtatgctgtgctggtcagcgcccttgtgttgatggccatggtcaagagaaaggatttc

SEQ ID NO: 154 - DNA, 936 bp, Artificial Sequence
  Nucleotide sequence encoding TCR, Donor HD5
atgggcacaaggttgttcttctatgtggccctttgtctcctgtggacaggacacatggatgctggaatcacccagagcccaagacacaaggtcacagagacaggaacaccagtgactctgagatgtcaccagactgagaaccaccgctatatgtactggtatcgacaagacccggggcatgggctgaggctgatccattactcatatggtgttaaagatactgacaaaggagaagtctcagatggctatagtgtctctagatcaaagacagaggatttcctcctcactctggagtccgctaccagctcccagacatctgtgtacttctgtgccatctcggtgggacagggggccctctacgagcagtacttcgggccgggcaccaggctcacggtcacagaggacctgaaaaacgtgttcccacccgaggtcgctgtgtttgagccatcagaagcagagatctcccacacccaaaaggccacactggtgtgcctggccacaggcttctaccccgaccacgtggagctgagctggtgggtgaatgggaaggaggtgcacagtggggtcagcacagacccgcagcccctcaaggagcagcccgccctcaatgactccagatactgcctgagcagccgcctgagggtctcggccaccttctggcagaacccccgcaaccacttccgctgtcaagtccagttctacgggctctcggagaatgacgagtggacccaggatagggccaaacctgtcacccagatcgtcagcgccgaggcctggggtagagcagactgtggcttcacctccgagtcttaccagcaaggggtcctgtctgccaccatcctctatgagatcttgctagggaaggccaccttgtatgccgtgctggtcagtgccctcgtgctgatggccatggtcaagagaaaggattccagaggc

SEQ ID NO: 155 - DNA, 933 bp, Artificial Sequence
  Nucleotide sequence encoding TCR, Donor HD5
atgggcttcaggctcctctgctgtgtggccttttgtctcctgggagcaggcccagtggattctggagtcacacaaaccccaaagcacctgatcacagcaactggacagcgagtgacgctgagatgctcccctaggtctggagacctctctgtgtactggtaccaacagagcctggaccagggcctccagttcctcattcagtattataatggagaagagagagcaaaaggaaacattcttgaacgattctccgcacaacagttccctgacttgcactctgaactaaacctgagctctctggagctgggggactcagctttgtatttctgtgccagcagcgtagctcgggacaggcggaactatggctacaccttcggttcggggaccaggttaaccgttgtagaggacctgaacaaggtgttcccacccgaggtcgctgtgtttgagccatcagaagcagagatctcccacacccaaaaggccacactggtgtgcctggccacaggcttcttccccgaccacgtggagctgagctggtgggtgaatgggaaggaggtgcacagtggggtcagcacggacccgcagcccctcaaggagcagcccgccctcaatgactccagatactgcctgagcagccgcctgagggtctcggccaccttctggcagaacccccgcaaccacttccgctgtcaagtccagttctacgggctctcggagaatgacgagtggacccaggatagggccaaacccgtcacccagatcgtcagcgccgaggcctggggtagagcagactgtggctttacctcggtgtcctaccagcaaggggtcctgtctgccaccatcctctatgagatcctgctagggaaggccaccctgtatgctgtgctggtcagcgcccttgtgttgatggccatggtcaagagaaaggatttc

SEQ ID NO: 156 - DNA, 939 bp, Artificial Sequence
  Nucleotide sequence encoding TCR, Donor HD5
atgggcttcaggctcctctgctgtgtggccttttgtctcctgggagcaggcccagtggattctggagtcacacaaaccccaaagcacctgatcacagcaactggacagcgagtgacgctgagatgctcccctaggtctggagacctctctgtgtactggtaccaacagagcctggaccagggcctccagttcctcattcagtattataatggagaagagagagcaaaaggaaacattcttgaacgattctccgcacaacagttccctgacttgcactctgaactaaacctgagctctctggagctgggggactcagctttgtatttctgtgccagcagcgtagctcgggacaggcggaactatggctacaccttcggttcggggaccaggttaaccgttgtagaggacctgaaaaacgtgttcccacccgaggtcgctgtgtttgagccatcagaagcagagatctcccacacccaaaaggccacactggtgtgcctggccacaggcttctaccccgaccacgtggagctgagctggtgggtgaatgggaaggaggtgcacagtggggtcagcacagacccgcagcccctcaaggagcagcccgccctcaatgactccagatactgcctgagcagccgcctgagggtctcggccaccttctggcagaacccccgcaaccacttccgctgtcaagtccagttctacgggctctcggagaatgacgagtggacccaggatagggccaaacctgtcacccagatcgtcagcgccgaggcctggggtagagcagactgtggcttcacctccgagtcttaccagcaaggggtcctgtctgccaccatcctctatgagatcttgctagggaaggccaccttgtatgccgtgctggtcagtgccctcgtgctgatggccatggtcaagagaaaggattccagaggc

SEQ ID NO: 157 - protein, 9 aa, Artificial Sequence
  nonamer peptide VLD
VLDFAPPGA

SEQ ID NO: 158 - protein, 9 aa, Artificial Sequence
  nonamer peptide PVL
PVLDFAPPG

SEQ ID NO: 159 - protein, 9 aa, Artificial Sequence
  nonamer peptide LDF
LDFAPPGAS

SEQ ID NO: 160 - protein, 271 aa, Artificial Sequence
  TCR amino acid sequence, Donor HD7
MTSIRAVFIFLWLQLDLVNGENVEQHPSTLSVQEGDSAVIKCTYSDSASNYFPWYKQELGKRPQLIIDIRSNVGEKKDQRIAVTLNKTAKHFSLHITETQPEDSAVYFCAVRTSYDKVIFGPGTSLSVIPNIQNPDPAVYQLRDSKSSDKSVCLFTDFDSQTNVSQSKDSDVYITDKTVLDMRSMDFKSNSAVAWSNKSDFACANAFNNSIIPEDTFFPSPESSCDVKLVEKSFETDTNLNFQNLSVIGFRILLLKVAGFNLLMTLRLWSS

SEQ ID NO: 161 - protein, 6 aa, Artificial Sequence
  TCR amino acid sequence, Donor HD7
DFQATT

SEQ ID NO: 162 - protein, 7 aa, Artificial Sequence
  TCR amino acid sequence, Donor HD7
SNEGSKA

SEQ ID NO: 163 - protein, 14 aa, Artificial Sequence
  TCR amino acid sequence, Donor HD7
CSARDSVSGNTIYF

SEQ ID NO: 164 - protein, 142 aa, Artificial Sequence
  TCR amino acid sequence, Donor HD7
MLLLLLLLGPGISLLLPGSLAGSGLGAVVSQHPSWVICKSGTSVKIECRSLDFQATTMFWYRQFPKQSLMLMATSNEGSKATYEQGVEKDKFLINHASLTLSTLTVTSAHPEDSSFYICSARDSVSGNTIYFGEGSWLTVVE

SEQ ID NO: 165 - protein, 318 aa, Artificial Sequence
  TCR amino acid sequence, Donor HD7
MLLLLLLLGPGISLLLPGSLAGSGLGAVVSQHPSWVICKSGTSVKIECRSLDFQATTMFWYRQFPKQSLMLMATSNEGSKATYEQGVEKDKFLINHASLTLSTLTVTSAHPEDSSFYICSARDSVSGNTIYFGEGSWLTVVEDLNKVFPPEVAVFEPSEAEISHTQKATLVCLATGFFPDHVELSWWVNGKEVHSGVSTDPQPLKEQPALNDSRYCLSSRLRVSATFWQNPRNHFRCQVQFYGLSENDEWTQDRAKPVTQIVSAEAWGRADCGFTSVSYQQGVLSATILYEILLGKATLYAVLVSALVLMAMVKRKDF

SEQ ID NO: 166 - protein, 320 aa, Artificial Sequence
  TCR amino acid sequence, Donor HD7
MLLLLLLLGPGISLLLPGSLAGSGLGAVVSQHPSWVICKSGTSVKIECRSLDFQATTMFWYRQFPKQSLMLMATSNEGSKATYEQGVEKDKFLINHASLTLSTLTVTSAHPEDSSFYICSARDSVSGNTIYFGEGSWLTVVEDLKNVFPPEVAVFEPSEAEISHTQKATLVCLATGFYPDHVELSWWVNGKEVHSGVSTDPQPLKEQPALNDSRYCLSSRLRVSATFWQNPRNHFRCQVQFYGLSENDEWTQDRAKPVTQIVSAEAWGRADCGFTSESYQQGVLSATILYEILLGKATLYAVLVSALVLMAMVKRKDSRG

SEQ ID NO: 167 - protein, 5 aa, Artificial Sequence
  TCR amino acid sequence, Donor HD7
SQVTM

SEQ ID NO: 168 - protein, 7 aa, Artificial Sequence
  TCR amino acid sequence, Donor HD7
ANQGSEA

SEQ ID NO: 169 - protein, 14 aa, Artificial Sequence
  TCR amino acid sequence, Donor HD7
CSVGGSGSYNEQFF

SEQ ID NO: 170 - protein, 131 aa, Artificial Sequence
  TCR amino acid sequence, Donor HD7
MLSLLLLLLGLGSVFSAVISQKPSRDICQRGTSLTIQCQVDSQVTMMFWYRQQPGQSLTLIATANQGSEATYESGFVIDKFPISRPNLTFSTLTVSNMSPEDSSIYLCSVGGSGSYNEQFFGPGTRLTVLE

SEQ ID NO: 171 - protein, 307 aa, Artificial Sequence
  TCR amino acid sequence, Donor HD7
MLSLLLLLLGLGSVFSAVISQKPSRDICQRGTSLTIQCQVDSQVTMMFWYRQQPGQSLTLIATANQGSEATYESGFVIDKFPISRPNLTFSTLTVSNMSPEDSSIYLCSVGGSGSYNEQFFGPGTRLTVLEDLNKVFPPEVAVFEPSEAEISHTQKATLVCLATGFFPDHVELSWWVNGKEVHSGVSTDPQPLKEQPALNDSRYCLSSRLRVSATFWQNPRNHFRCQVQFYGLSENDEWTQDRAKPVTQIVSAEAWGRADCGFTSVSYQQGVLSATILYEILLGKATLYAVLVSALVLMAMVKRKDF

SEQ ID NO: 172 - protein, 309 aa, Artificial Sequence
  TCR amino acid sequence, Donor HD7
MLSLLLLLLGLGSVFSAVISQKPSRDICQRGTSLTIQCQVDSQVTMMFWYRQQPGQSLTLIATANQGSEATYESGFVIDKFPISRPNLTFSTLTVSNMSPEDSSIYLCSVGGSGSYNEQFFGPGTRLTVLEDLKNVFPPEVAVFEPSEAEISHTQKATLVCLATGFYPDHVELSWWVNGKEVHSGVSTDPQPLKEQPALNDSRYCLSSRLRVSATFWQNPRNHFRCQVQFYGLSENDEWTQDRAKPVTQIVSAEAWGRADCGFTSESYQQGVLSATILYEILLGKATLYAVLVSALVLMAMVKRKDSRG

SEQ ID NO: 173 - protein, 5 aa, Artificial Sequence
  TCR amino acid sequence, Donor HD8
VGISA

SEQ ID NO: 174 - protein, 5 aa, Artificial Sequence
  TCR amino acid sequence, Donor HD8
LSSGK

SEQ ID NO: 175 - protein, 11 aa, Artificial Sequence
  TCR amino acid sequence, Donor HD8
CAVTVGNKLVF

SEQ ID NO: 176 - protein, 130 aa, Artificial Sequence
  TCR amino acid sequence, Donor HD8
MVKIRQFLLAILWLQLSCVSAAKNEVEQSPQNLTAQEGEFITINCSYSVGISALHWLQQHPGGGIVSLFMLSSGKKKHGRLIATINIQEKHSSLHITASHPRDSAVYICAVTVGNKLVFGAGTILRVKSY

SEQ ID NO: 177 - protein, 270 aa, Artificial Sequence
  TCR amino acid sequence, Donor HD8
MVKIRQFLLAILWLQLSCVSAAKNEVEQSPQNLTAQEGEFITINCSYSVGISALHWLQQHPGGGIVSLFMLSSGKKKHGRLIATINIQEKHSSLHITASHPRDSAVYICAVTVGNKLVFGAGTILRVKSYIQNPDPAVYQLRDSKSSDKSVCLFTDFDSQTNVSQSKDSDVYITDKTVLDMRSMDFKSNSAVAWSNKSDFACANAFNNSIIPEDTFFPSPESSCDVKLVEKSFETDTNLNFQNLSVIGFRILLLKVAGFNLLMTLRLWSS

SEQ ID NO: 178 - protein, 5 aa, Artificial Sequence
  TCR amino acid sequence, Donor HD8
MNHNS

SEQ ID NO: 179 - protein, 6 aa, Artificial Sequence
  TCR amino acid sequence, Donor HD8
SASEGT

SEQ ID NO: 180 - protein, 11 aa, Artificial Sequence
  TCR amino acid sequence, Donor HD8
CASRGWREQFF

SEQ ID NO: 181 - protein, 130 aa, Artificial Sequence
  TCR amino acid sequence, Donor HD8
MSIGLLCCVAFSLLWASPVNAGVTQTPKFQVLKTGQSMTLQCAQDMNHNSMYWYRQDPGMGLRLIYYSASEGTTDKGEVPNGYNVSRLNKREFSLRLESAAPSQTSVYFCASRGWREQFFGPGTRLTVLE

SEQ ID NO: 182 - protein, 306 aa, Artificial Sequence
  TCR amino acid sequence, Donor HD8
MSIGLLCCVAFSLLWASPVNAGVTQTPKFQVLKTGQSMTLQCAQDMNHNSMYWYRQDPGMGLRLIYYSASEGTTDKGEVPNGYNVSRLNKREFSLRLESAAPSQTSVYFCASRGWREQFFGPGTRLTVLEDLNKVFPPEVAVFEPSEAEISHTQKATLVCLATGFFPDHVELSWWVNGKEVHSGVSTDPQPLKEQPALNDSRYCLSSRLRVSATFWQNPRNHFRCQVQFYGLSENDEWTQDRAKPVTQIVSAEAWGRADCGFTSVSYQQGVLSATILYEILLGKATLYAVLVSALVLMAMVKRKDF

SEQ ID NO: 183 - protein, 308 aa, Artificial Sequence
  TCR amino acid sequence, Donor HD8
MSIGLLCCVAFSLLWASPVNAGVTQTPKFQVLKTGQSMTLQCAQDMNHNSMYWYRQDPGMGLRLIYYSASEGTTDKGEVPNGYNVSRLNKREFSLRLESAAPSQTSVYFCASRGWREQFFGPGTRLTVLEDLKNVFPPEVAVFEPSEAEISHTQKATLVCLATGFYPDHVELSWWVNGKEVHSGVSTDPQPLKEQPALNDSRYCLSSRLRVSATFWQNPRNHFRCQVQFYGLSENDEWTQDRAKPVTQIVSAEAWGRADCGFTSESYQQGVLSATILYEILLGKATLYAVLVSALVLMAMVKRKDSRG

SEQ ID NO: 184 - protein, 5 aa, Artificial Sequence
  TCR amino acid sequence, Donor HD9
VGISA

SEQ ID NO: 185 - protein, 5 aa, Artificial Sequence
  TCR amino acid sequence, Donor HD9
LSSGK

SEQ ID NO: 186 - protein, 13 aa, Artificial Sequence
  TCR amino acid sequence, Donor HD9
CAARSYNTDKLIF

SEQ ID NO: 187 - protein, 132 aa, Artificial Sequence
  TCR amino acid sequence, Donor HD9
MVKIRQFLLAILWLQLSCVSAAKNEVEQSPQNLTAQEGEFITINCSYSVGISALHWLQQHPGGGIVSLFMLSSGKKKHGRLIATINIQEKHSSLHITASHPRDSAVYICAARSYNTDKLIFGTGTRLQVFPN

SEQ ID NO: 188 - protein, 272 aa, Artificial Sequence
  TCR amino acid sequence, Donor HD9
MVKIRQFLLAILWLQLSCVSAAKNEVEQSPQNLTAQEGEFITINCSYSVGISALHWLQQHPGGGIVSLFMLSSGKKKHGRLIATINIQEKHSSLHITASHPRDSAVYICAARSYNTDKLIFGTGTRLQVFPNIQNPDPAVYQLRDSKSSDKSVCLFTDFDSQTNVSQSKDSDVYITDKTVLDMRSMDFKSNSAVAWSNKSDFACANAFNNSIIPEDTFFPSPESSCDVKLVEKSFETDTNLNFQNLSVIGFRILLLKVAGFNLLMTLRLWSS

SEQ ID NO: 189 - protein, 6 aa, Artificial Sequence
  TCR amino acid sequence, Donor HD9
NSMFDY

SEQ ID NO: 190 - protein, 7 aa, Artificial Sequence
  TCR amino acid sequence, Donor HD9
ISSIKDK

SEQ ID NO: 191 - protein, 12 aa, Artificial Sequence
  TCR amino acid sequence, Donor HD9
CAASYNNARLMF

SEQ ID NO: 192 - protein, 138 aa, Artificial Sequence
  TCR amino acid sequence, Donor HD9
MAMLLGASVLILWLQPDWVNSQQKNDDQQVKQNSPSLSVQEGRISILNCDYTNSMFDYFLWYKKYPAEGPTFLISISSIKDKNEDGRFTVFLNKSAKHLSLHIVPSQPGDSAVYFCAASYNNARLMFGDGTQLVVKPN

SEQ ID NO: 193 - protein, 278 aa, Artificial Sequence
  TCR amino acid sequence, Donor HD9
MAMLLGASVLILWLQPDWVNSQQKNDDQQVKQNSPSLSVQEGRISILNCDYTNSMFDYFLWYKKYPAEGPTFLISISSIKDKNEDGRFTVFLNKSAKHLSLHIVPSQPGDSAVYFCAASYNNARLMFGDGTQLVVKPNIQNPDPAVYQLRDSKSSDKSVCLFTDFDSQTNVSQSKDSDVYITDKTVLDMRSMDFKSNSAVAWSNKSDFACANAFNNSIIPEDTFFPSPESSCDVKLVEKSFETDTNLNFQNLSVIGFRILLLKVAGFNLLMTLRLWSS

SEQ ID NO: 194 - protein, 5 aa, Artificial Sequence
  TCR amino acid sequence, Donor HD9
SGHTS

SEQ ID NO: 195 - protein, 6 aa, Artificial Sequence
  TCR amino acid sequence, Donor HD9
YDEGEE

SEQ ID NO: 196 - protein, 13 aa, Artificial Sequence
  TCR amino acid sequence, Donor HD9
CASSWGYQETQYF

SEQ ID NO: 197 - protein, 132 aa, Artificial Sequence
  TCR amino acid sequence, Donor HD9
MGPRLLFWALLCLLGTGPVEAGVTQSPTHLIKTRGQQATLRCSPISGHTSVYWYQQALGLGLQFLLWYDEGEERNRGNFPPRFSGRQFPNYSSELNVNALELEDSALYLCASSWGYQETQYFGPGTRLLVLE

SEQ ID NO: 198 - protein, 308 aa, Artificial Sequence
  TCR amino acid sequence, Donor HD9
MGPRLLFWALLCLLGTGPVEAGVTQSPTHLIKTRGQQATLRCSPISGHTSVYWYQQALGLGLQFLLWYDEGEERNRGNFPPRFSGRQFPNYSSELNVNALELEDSALYLCASSWGYQETQYFGPGTRLLVLEDLNKVFPPEVAVFEPSEAEISHTQKATLVCLATGFFPDHVELSWWVNGKEVHSGVSTDPQPLKEQPALNDSRYCLSSRLRVSATFWQNPRNHFRCQVQFYGLSENDEWTQDRAKPVTQIVSAEAWGRADCGFTSVSYQQGVLSATILYEILLGKATLYAVLVSALVLMAMVKRKDF

SEQ ID NO: 199 - protein, 310 aa, Artificial Sequence
  TCR amino acid sequence, Donor HD9
MGPRLLFWALLCLLGTGPVEAGVTQSPTHLIKTRGQQATLRCSPISGHTSVYWYQQALGLGLQFLLWYDEGEERNRGNFPPRFSGRQFPNYSSELNVNALELEDSALYLCASSWGYQETQYFGPGTRLLVLEDLKNVFPPEVAVFEPSEAEISHTQKATLVCLATGFYPDHVELSWWVNGKEVHSGVSTDPQPLKEQPALNDSRYCLSSRLRVSATFWQNPRNHFRCQVQFYGLSENDEWTQDRAKPVTQIVSAEAWGRADCGFTSESYQQGVLSATILYEILLGKATLYAVLVSALVLMAMVKRKDSRG

SEQ ID NO: 200 - protein, 5 aa, Artificial Sequence
  TCR amino acid sequence, Donor HD9
KGHSH

SEQ ID NO: 201 - protein, 6 aa, Artificial Sequence
  TCR amino acid sequence, Donor HD9
LQKENI

SEQ ID NO: 202 - protein, 15 aa, Artificial Sequence
  TCR amino acid sequence, Donor HD9
CASSPTGGEYYGYTF

SEQ ID NO: 203 - protein, 135 aa, Artificial Sequence
  TCR amino acid sequence, Donor HD9
MDTRVLCCAVICLLGAGLSNAGVMQNPRHLVRRRGQEARLRCSPMKGHSHVYWYRQLPEEGLKFMVYLQKENIIDESGMPKERFSAEFPKEGPSILRIQQVVRGDSAAYFCASSPTGGEYYGYTFGSGTRLTVVE

SEQ ID NO: 204 - protein, 311 aa, Artificial Sequence
  TCR amino acid sequence, Donor HD9
MDTRVLCCAVICLLGAGLSNAGVMQNPRHLVRRRGQEARLRCSPMKGHSHVYWYRQLPEEGLKFMVYLQKENIIDESGMPKERFSAEFPKEGPSILRIQQVVRGDSAAYFCASSPTGGEYYGYTFGSGTRLTVVEDLNKVFPPEVAVFEPSEAEISHTQKATLVCLATGFFPDHVELSWWVNGKEVHSGVSTDPQPLKEQPALNDSRYCLSSRLRVSATFWQNPRNHFRCQVQFYGLSENDEWTQDRAKPVTQIVSAEAWGRADCGFTSVSYQQGVLSATILYEILLGKATLYAVLVSALVLMAMVKRKDF

SEQ ID NO: 205 - protein, 313 aa, Artificial Sequence
  TCR amino acid sequence, Donor HD9
MDTRVLCCAVICLLGAGLSNAGVMQNPRHLVRRRGQEARLRCSPMKGHSHVYWYRQLPEEGLKFMVYLQKENIIDESGMPKERFSAEFPKEGPSILRIQQVVRGDSAAYFCASSPTGGEYYGYTFGSGTRLTVVEDLKNVFPPEVAVFEPSEAEISHTQKATLVCLATGFYPDHVELSWWVNGKEVHSGVSTDPQPLKEQPALNDSRYCLSSRLRVSATFWQNPRNHFRCQVQFYGLSENDEWTQDRAKPVTQIVSAEAWGRADCGFTSESYQQGVLSATILYEILLGKATLYAVLVSALVLMAMVKRKDSRG

SEQ ID NO: 206 - protein, 5 aa, Artificial Sequence
  TCR amino acid sequence, Donor HD9
MNHEY

SEQ ID NO: 207 - protein, 6 aa, Artificial Sequence
  TCR amino acid sequence, Donor HD9
SVGAGI

SEQ ID NO: 208 - protein, 22 aa, Artificial Sequence
  TCR amino acid sequence, Donor HD9
CASSSYPLRTGRYNSYNSPLHF

SEQ ID NO: 209 - protein, 141 aa, Artificial Sequence
  TCR amino acid sequence, Donor HD9
MSIGLLCCAALSLLWAGPVNAGVTQTPKFQVLKTGQSMTLQCAQDMNHEYMSWYRQDPGMGLRLIHYSVGAGITDQGEVPNGYNVSRSTTEDFPLRLLSAAPSQTSVYFCASSSYPLRTGRYNSYNSPLHFGNGTRLTVTE

SEQ ID NO: 210 - protein, 317 aa, Artificial Sequence
  TCR amino acid sequence, Donor HD9
MSIGLLCCAALSLLWAGPVNAGVTQTPKFQVLKTGQSMTLQCAQDMNHEYMSWYRQDPGMGLRLIHYSVGAGITDQGEVPNGYNVSRSTTEDFPLRLLSAAPSQTSVYFCASSSYPLRTGRYNSYNSPLHFGNGTRLTVTEDLNKVFPPEVAVFEPSEAEISHTQKATLVCLATGFFPDHVELSWWVNGKEVHSGVSTDPQPLKEQPALNDSRYCLSSRLRVSATFWQNPRNHFRCQVQFYGLSENDEWTQDRAKPVTQIVSAEAWGRADCGFTSVSYQQGVLSATILYEILLGKATLYAVLVSALVLMAMVKRKDF

SEQ ID NO: 211 - protein, 319 aa, Artificial Sequence
  TCR amino acid sequence, Donor HD9
MSIGLLCCAALSLLWAGPVNAGVTQTPKFQVLKTGQSMTLQCAQDMNHEYMSWYRQDPGMGLRLIHYSVGAGITDQGEVPNGYNVSRSTTEDFPLRLLSAAPSQTSVYFCASSSYPLRTGRYNSYNSPLHFGNGTRLTVTEDLKNVFPPEVAVFEPSEAEISHTQKATLVCLATGFYPDHVELSWWVNGKEVHSGVSTDPQPLKEQPALNDSRYCLSSRLRVSATFWQNPRNHFRCQVQFYGLSENDEWTQDRAKPVTQIVSAEAWGRADCGFTSESYQQGVLSATILYEILLGKATLYAVLVSALVLMAMVKRKDSRG

SEQ ID NO: 212 - protein, 6 aa, Artificial Sequence
  TCR amino acid sequence, Donor HD10
NSMFDY

SEQ ID NO: 213 - protein, 7 aa, Artificial Sequence
  TCR amino acid sequence, Donor HD10
ISSIKDK

SEQ ID NO: 214 - protein, 13 aa, Artificial Sequence
  TCR amino acid sequence, Donor HD10
CAASGGRDDKIIF

SEQ ID NO: 215 - protein, 139 aa, Artificial Sequence
  TCR amino acid sequence, Donor HD10
MAMLLGASVLILWLQPDWVNSQQKNDDQQVKQNSPSLSVQEGRISILNCDYTNSMFDYFLWYKKYPAEGPTFLISISSIKDKNEDGRFTVFLNKSAKHLSLHIVPSQPGDSAVYFCAASGGRDDKIIFGKGTRLHILPN

SEQ ID NO: 216 - protein, 279 aa, Artificial Sequence
  TCR amino acid sequence, Donor HD10
MAMLLGASVLILWLQPDWVNSQQKNDDQQVKQNSPSLSVQEGRISILNCDYTNSMFDYFLWYKKYPAEGPTFLISISSIKDKNEDGRFTVFLNKSAKHLSLHIVPSQPGDSAVYFCAASGGRDDKIIFGKGTRLHILPNIQNPDPAVYQLRDSKSSDKSVCLFTDFDSQTNVSQSKDSDVYITDKTVLDMRSMDFKSNSAVAWSNKSDFACANAFNNSIIPEDTFFPSPESSCDVKLVEKSFETDTNLNFQNLSVIGFRILLLKVAGFNLLMTLRLWSS

SEQ ID NO: 217 - protein, 5 aa, Artificial Sequence
  TCR amino acid sequence, Donor HD10
MNHEY

SEQ ID NO: 218 - protein, 6 aa, Artificial Sequence
  TCR amino acid sequence, Donor HD10
SVGAGI

SEQ ID NO: 219 - protein, 16 aa, Artificial Sequence
  TCR amino acid sequence, Donor HD10
CASSYSRTESTDTQYF

SEQ ID NO: 220 - protein, 135 aa, Artificial Sequence
  TCR amino acid sequence, Donor HD10
MSIGLLCCAALSLLWAGPVNAGVTQTPKFQVLKTGQSMTLQCAQDMNHEYMSWYRQDPGMGLRLIHYSVGAGITDQGEVPNGYNVSRSTTEDFPLRLLSAAPSQTSVYFCASSYSRTESTDTQYFGPGTRLTVLE

SEQ ID NO: 221 - protein, 311 aa, Artificial Sequence
  TCR amino acid sequence, Donor HD10
MSIGLLCCAALSLLWAGPVNAGVTQTPKFQVLKTGQSMTLQCAQDMNHEYMSWYRQDPGMGLRLIHYSVGAGITDQGEVPNGYNVSRSTTEDFPLRLLSAAPSQTSVYFCASSYSRTESTDTQYFGPGTRLTVLEDLNKVFPPEVAVFEPSEAEISHTQKATLVCLATGFFPDHVELSWWVNGKEVHSGVSTDPQPLKEQPALNDSRYCLSSRLRVSATFWQNPRNHFRCQVQFYGLSENDEWTQDRAKPVTQIVSAEAWGRADCGFTSVSYQQGVLSATILYEILLGKATLYAVLVSALVLMAMVKRKDF

SEQ ID NO: 222 - protein, 313 aa, Artificial Sequence
  TCR amino acid sequence, Donor HD10
MSIGLLCCAALSLLWAGPVNAGVTQTPKFQVLKTGQSMTLQCAQDMNHEYMSWYRQDPGMGLRLIHYSVGAGITDQGEVPNGYNVSRSTTEDFPLRLLSAAPSQTSVYFCASSYSRTESTDTQYFGPGTRLTVLEDLKNVFPPEVAVFEPSEAEISHTQKATLVCLATGFYPDHVELSWWVNGKEVHSGVSTDPQPLKEQPALNDSRYCLSSRLRVSATFWQNPRNHFRCQVQFYGLSENDEWTQDRAKPVTQIVSAEAWGRADCGFTSESYQQGVLSATILYEILLGKATLYAVLVSALVLMAMVKRKDSRG

SEQ ID NO: 223 - DNA, 828 bp, Artificial Sequence
  Nucleotide sequence encoding TCR, Donor HD6
atggccatgctcctgggggcatcagtgctgattctgtggcttcagccagactgggtaaacagtcaacagaagaatgatgaccagcaagttaagcaaaattcaccatccctgagcgtccaggaaggaagaatttctattctgaactgtgactatactaacagcatgtttgattatttcctatggtacaaaaaataccctgctgaaggtcctacattcctgatatctataagttccattaaggataaaaatgaagatggaagattcactgtcttcttaaacaaaagtgccaagcacctctctctgcacattgtgccctcccagcctggagactctgcagtgtacttctgtgcagcaaacaatgccagactcatgtttggagatggaactcagctggtggtgaagcccaatatccagaaccctgaccctgccgtgtaccagctgagagactctaaatccagtgacaagtctgtctgcctattcaccgattttgattctcaaacaaatgtgtcacaaagtaaggattctgatgtgtatatcacagacaaaactgtgctagacatgaggtctatggacttcaagagcaacagtgctgtggcctggagcaacaaatctgactttgcatgtgcaaacgccttcaacaacagcattattccagaagacaccttcttccccagcccagaaagttcctgtgatgtcaagctggtcgagaaaagctttgaaacagatacgaacctaaactttcaaaacctgtcagtgattgggttccgaatcctcctcctgaaagtggccgggtttaatctgctcatgacgctgcggctgtggtccagc

SEQ ID NO: 224 - DNA, 927 bp, Artificial Sequence
  Nucleotide sequence encoding TCR, Donor HD6
atggactcctggaccttctgctgtgtgtccctttgcatcctggtagcgaagcatacagatgctggagttatccagtcaccccgccatgaggtgacagagatgggacaagaagtgactctgagatgtaaaccaatttcaggccacaactcccttttctggtacagacagaccatgatgcggggactggagttgctcatttactttaacaacaacgttccgatagatgattcagggatgcccgaggatcgattctcagctaagatgcctaatgcatcattctccactctgaagatccagccctcagaacccagggactcagctgtgtacttctgtgccagcagtgataccagggcccgggagcagttcttcgggccagggacacggctcaccgtgctagaggacctgaacaaggtgttcccacccgaggtcgctgtgtttgagccatcagaagcagagatctcccacacccaaaaggccacactggtgtgcctggccacaggcttcttccccgaccacgtggagctgagctggtgggtgaatgggaaggaggtgcacagtggggtcagcacggacccgcagcccctcaaggagcagcccgccctcaatgactccagatactgcctgagcagccgcctgagggtctcggccaccttctggcagaacccccgcaaccacttccgctgtcaagtccagttctacgggctctcggagaatgacgagtggacccaggatagggccaaacccgtcacccagatcgtcagcgccgaggcctggggtagagcagactgtggctttacctcggtgtcctaccagcaaggggtcctgtctgccaccatcctctatgagatcctgctagggaaggccaccctgtatgctgtgctggtcagcgcccttgtgttgatggccatggtcaagagaaaggatttc

SEQ ID NO: 225 - DNA, 933 bp, Artificial Sequence
  Nucleotide sequence encoding TCR, Donor HD6
atggactcctggaccttctgctgtgtgtccctttgcatcctggtagcgaagcatacagatgctggagttatccagtcaccccgccatgaggtgacagagatgggacaagaagtgactctgagatgtaaaccaatttcaggccacaactcccttttctggtacagacagaccatgatgcggggactggagttgctcatttactttaacaacaacgttccgatagatgattcagggatgcccgaggatcgattctcagctaagatgcctaatgcatcattctccactctgaagatccagccctcagaacccagggactcagctgtgtacttctgtgccagcagtgataccagggcccgggagcagttcttcgggccagggacacggctcaccgtgctagaggacctgaaaaacgtgttcccacccgaggtcgctgtgtttgagccatcagaagcagagatctcccacacccaaaaggccacactggtgtgcctggccacaggcttctaccccgaccacgtggagctgagctggtgggtgaatgggaaggaggtgcacagtggggtcagcacagacccgcagcccctcaaggagcagcccgccctcaatgactccagatactgcctgagcagccgcctgagggtctcggccaccttctggcagaacccccgcaaccacttccgctgtcaagtccagttctacgggctctcggagaatgacgagtggacccaggatagggccaaacctgtcacccagatcgtcagcgccgaggcctggggtagagcagactgtggcttcacctccgagtcttaccagcaaggggtcctgtctgccaccatcctctatgagatcttgctagggaaggccaccttgtatgccgtgctggtcagtgccctcgtgctgatggccatggtcaagagaaaggattccagaggc

SEQ ID NO: 226 - DNA, 816 bp, Artificial Sequence
  Nucleotide sequence encoding TCR, Donor HD7
atgaagacatttgctggattttcgttcctgtttttgtggctgcagctggactgtatgagtagaggagaggatgtggagcagagtcttttcctgagtgtccgagagggagacagctccgttataaactgcacttacacagacagctcctccacctacttatactggtataagcaagaacctggagcaggtctccagttgctgacgtatattttttcaaatatggacatgaaacaagaccaaagactcactgttctattgaataaaaaggataaacatctgtctctgcgcattgcagacacccagactggggactcagctatctacttctgtgcagagaggcttaacaccgacaagctcatctttgggactgggaccagattacaagtctttccaaatatccagaaccctgaccctgccgtgtaccagctgagagactctaaatccagtgacaagtctgtctgcctattcaccgattttgattctcaaacaaatgtgtcacaaagtaaggattctgatgtgtatatcacagacaaaactgtgctagacatgaggtctatggacttcaagagcaacagtgctgtggcctggagcaacaaatctgactttgcatgtgcaaacgccttcaacaacagcattattccagaagacaccttcttccccagcccagaaagttcctgtgatgtcaagctggtcgagaaaagctttgaaacagatacgaacctaaactttcaaaacctgtcagtgattgggttccgaatcctcctcctgaaagtggccgggtttaatctgctcatgacgctgcggctgtggtccagc

SEQ ID NO: 227 - DNA, 813 bp, Artificial Sequence
  Nucleotide sequence encoding TCR, Donor HD7
atgaagaggatattgggagctctgctggggctcttgagtgcccaggtttgctgtgtgagaggaatacaagtggagcagagtcctccagacctgattctccaggagggagccaattccacgctgcggtgcaatttttctgactctgtgaacaatttgcagtggtttcatcaaaacccttggggacagctcatcaacctgttttacattccctcagggacaaaacagaatggaagattaagcgccacgactgtcgctacggaacgctacagcttattgtacatttcctcttcccagaccacagactcaggcgtttatttctgtgctgtggaggcaactgacagctgggggaaattgcagtttggagcagggacccaggttgtggtcaccccagatatccagaaccctgaccctgccgtgtaccagctgagagactctaaatccagtgacaagtctgtctgcctattcaccgattttgattctcaaacaaatgtgtcacaaagtaaggattctgatgtgtatatcacagacaaaactgtgctagacatgaggtctatggacttcaagagcaacagtgctgtggcctggagcaacaaatctgactttgcatgtgcaaacgccttcaacaacagcattattccagaagacaccttcttccccagcccagaaagttcctgtgatgtcaagctggtcgagaaaagctttgaaacagatacgaacctaaactttcaaaacctgtcagtgattgggttccgaatcctcctcctgaaagtggccgggtttaatctgctcatgacgctgcggctgtggtccagc

SEQ ID NO: 228 - DNA, 813 bp, Artificial Sequence
  Nucleotide sequence encoding TCR, Donor HD7
atgacatccattcgagctgtatttatattcctgtggctgcagctggacttggtgaatggagagaatgtggagcagcatccttcaaccctgagtgtccaggagggagacagcgctgttatcaagtgtacttattcagacagtgcctcaaactacttcccttggtataagcaagaacttggaaaaagacctcagcttattatagacattcgttcaaatgtgggcgaaaagaaagaccaacgaattgctgttacattgaacaagacagccaaacatttctccctgcacatcacagagacccaacctgaagactcggctgtctacttctgtgcagtacgaacctcctacgacaaggtgatatttgggccagggacaagcttatcagtcattccaaatatccagaaccctgaccctgccgtgtaccagctgagagactctaaatccagtgacaagtctgtctgcctattcaccgattttgattctcaaacaaatgtgtcacaaagtaaggattctgatgtgtatatcacagacaaaactgtgctagacatgaggtctatggacttcaagagcaacagtgctgtggcctggagcaacaaatctgactttgcatgtgcaaacgccttcaacaacagcattattccagaagacaccttcttccccagcccagaaagttcctgtgatgtcaagctggtcgagaaaagctttgaaacagatacgaacctaaactttcaaaacctgtcagtgattgggttccgaatcctcctcctgaaagtggccgggtttaatctgctcatgacgctgcggctgtggtccagc

SEQ ID NO: 229 - DNA, 954 bp, Artificial Sequence
  Nucleotide sequence encoding TCR, Donor HD7
atgctgctgcttctgctgcttctggggccaggtataagcctccttctacctgggagcttggcaggctccgggcttggtgctgtcgtctctcaacatccgagctgggttatctgtaagagtggaacctctgtgaagatcgagtgccgttccctggactttcaggccacaactatgttttggtatcgtcagttcccgaaacagagtctcatgctgatggcaacttccaatgagggctccaaggccacatacgagcaaggcgtcgagaaggacaagtttctcatcaaccatgcaagcctgaccttgtccactctgacagtgaccagtgcccatcctgaagacagcagcttctacatctgcagtgctagggacagtgtgtctggaaacaccatatattttggagagggaagttggctcactgttgtagaggacctgaacaaggtgttcccacccgaggtcgctgtgtttgagccatcagaagcagagatctcccacacccaaaaggccacactggtgtgcctggccacaggcttcttccccgaccacgtggagctgagctggtgggtgaatgggaaggaggtgcacagtggggtcagcacggacccgcagcccctcaaggagcagcccgccctcaatgactccagatactgcctgagcagccgcctgagggtctcggccaccttctggcagaacccccgcaaccacttccgctgtcaagtccagttctacgggctctcggagaatgacgagtggacccaggatagggccaaacccgtcacccagatcgtcagcgccgaggcctggggtagagcagactgtggctttacctcggtgtcctaccagcaaggggtcctgtctgccaccatcctctatgagatcctgctagggaaggccaccctgtatgctgtgctggtcagcgcccttgtgttgatggccatggtcaagagaaaggatttc

SEQ ID NO: 230 - DNA, 960 bp, Artificial Sequence
  Nucleotide sequence encoding TCR, Donor HD7
atgctgctgcttctgctgcttctggggccaggtataagcctccttctacctgggagcttggcaggctccgggcttggtgctgtcgtctctcaacatccgagctgggttatctgtaagagtggaacctctgtgaagatcgagtgccgttccctggactttcaggccacaactatgttttggtatcgtcagttcccgaaacagagtctcatgctgatggcaacttccaatgagggctccaaggccacatacgagcaaggcgtcgagaaggacaagtttctcatcaaccatgcaagcctgaccttgtccactctgacagtgaccagtgcccatcctgaagacagcagcttctacatctgcagtgctagggacagtgtgtctggaaacaccatatattttggagagggaagttggctcactgttgtagaggacctgaaaaacgtgttcccacccgaggtcgctgtgtttgagccatcagaagcagagatctcccacacccaaaaggccacactggtgtgcctggccacaggcttctaccccgaccacgtggagctgagctggtgggtgaatgggaaggaggtgcacagtggggtcagcacagacccgcagcccctcaaggagcagcccgccctcaatgactccagatactgcctgagcagccgcctgagggtctcggccaccttctggcagaacccccgcaaccacttccgctgtcaagtccagttctacgggctctcggagaatgacgagtggacccaggatagggccaaacctgtcacccagatcgtcagcgccgaggcctggggtagagcagactgtggcttcacctccgagtcttaccagcaaggggtcctgtctgccaccatcctctatgagatcttgctagggaaggccaccttgtatgccgtgctggtcagtgccctcgtgctgatggccatggtcaagagaaaggattccagaggc

SEQ ID NO: 231 - DNA, 921 bp, Artificial Sequence
  Nucleotide sequence encoding TCR, Donor HD7
atgctgagtcttctgctccttctcctgggactaggctctgtgttcagtgctgtcatctctcaaaagccaagcagggatatctgtcaacgtggaacctccctgacgatccagtgtcaagtcgatagccaagtcaccatgatgttctggtaccgtcagcaacctggacagagcctgacactgatcgcaactgcaaatcagggctctgaggccacatatgagagtggatttgtcattgacaagtttcccatcagccgcccaaacctaacattctcaactctgactgtgagcaacatgagccctgaagacagcagcatatatctctgcagcgttgggggtagcgggagttacaatgagcagttcttcgggccagggacacggctcaccgtgctagaggacctgaacaaggtgttcccacccgaggtcgctgtgtttgagccatcagaagcagagatctcccacacccaaaaggccacactggtgtgcctggccacaggcttcttccccgaccacgtggagctgagctggtgggtgaatgggaaggaggtgcacagtggggtcagcacggacccgcagcccctcaaggagcagcccgccctcaatgactccagatactgcctgagcagccgcctgagggtctcggccaccttctggcagaacccccgcaaccacttccgctgtcaagtccagttctacgggctctcggagaatgacgagtggacccaggatagggccaaacccgtcacccagatcgtcagcgccgaggcctggggtagagcagactgtggctttacctcggtgtcctaccagcaaggggtcctgtctgccaccatcctctatgagatcctgctagggaaggccaccctgtatgctgtgctggtcagcgcccttgtgttgatggccatggtcaagagaaaggatttc

SEQ ID NO: 232 - DNA, 927 bp, Artificial Sequence
  Nucleotide sequence encoding TCR, Donor HD7
atgctgagtcttctgctccttctcctgggactaggctctgtgttcagtgctgtcatctctcaaaagccaagcagggatatctgtcaacgtggaacctccctgacgatccagtgtcaagtcgatagccaagtcaccatgatgttctggtaccgtcagcaacctggacagagcctgacactgatcgcaactgcaaatcagggctctgaggccacatatgagagtggatttgtcattgacaagtttcccatcagccgcccaaacctaacattctcaactctgactgtgagcaacatgagccctgaagacagcagcatatatctctgcagcgttgggggtagcgggagttacaatgagcagttcttcgggccagggacacggctcaccgtgctagaggacctgaaaaacgtgttcccacccgaggtcgctgtgtttgagccatcagaagcagagatctcccacacccaaaaggccacactggtgtgcctggccacaggcttctaccccgaccacgtggagctgagctggtgggtgaatgggaaggaggtgcacagtggggtcagcacagacccgcagcccctcaaggagcagcccgccctcaatgactccagatactgcctgagcagccgcctgagggtctcggccaccttctggcagaacccccgcaaccacttccgctgtcaagtccagttctacgggctctcggagaatgacgagtggacccaggatagggccaaacctgtcacccagatcgtcagcgccgaggcctggggtagagcagactgtggcttcacctccgagtcttaccagcaaggggtcctgtctgccaccatcctctatgagatcttgctagggaaggccaccttgtatgccgtgctggtcagtgccctcgtgctgatggccatggtcaagagaaaggattccagaggc

SEQ ID NO: 233 - DNA, 810 bp, Artificial Sequence
  Nucleotide sequence encoding TCR, Donor HD8
atggtgaagatccggcaatttttgttggctattttgtggcttcagctaagctgtgtaagtgccgccaaaaatgaagtggagcagagtcctcagaacctgactgcccaggaaggagaatttatcacaatcaactgcagttactcggtaggaataagtgccttacactggctgcaacagcatccaggaggaggcattgtttccttgtttatgctgagctcagggaagaagaagcatggaagattaattgccacaataaacatacaggaaaagcacagctccctgcacatcacagcctcccatcccagagactctgccgtctacatctgtgctgtcacagtcggaaacaaactggtctttggcgcaggaaccattctgagagtcaagtcctatatccagaaccctgaccctgccgtgtaccagctgagagactctaaatccagtgacaagtctgtctgcctattcaccgattttgattctcaaacaaatgtgtcacaaagtaaggattctgatgtgtatatcacagacaaaactgtgctagacatgaggtctatggacttcaagagcaacagtgctgtggcctggagcaacaaatctgactttgcatgtgcaaacgccttcaacaacagcattattccagaagacaccttcttccccagcccagaaagttcctgtgatgtcaagctggtcgagaaaagctttgaaacagatacgaacctaaactttcaaaacctgtcagtgattgggttccgaatcctcctcctgaaagtggccgggtttaatctgctcatgacgctgcggctgtggtccagc

SEQ ID NO: 234 - DNA, 918 bp, Artificial Sequence
  Nucleotide sequence encoding TCR, Donor HD8
atgagcatcgggctcctgtgctgtgtggccttttctctcctgtgggcaagtccagtgaatgctggtgtcactcagaccccaaaattccaggtcctgaagacaggacagagcatgacactgcagtgtgcccaggatatgaaccataactccatgtactggtatcgacaagacccaggcatgggactgaggctgatttattactcagcttctgagggtaccactgacaaaggagaagtccccaatggctacaatgtctccagattaaacaaacgggagttctcgctcaggctggagtcggctgctccctcccagacatctgtgtacttctgtgccagcagggggtggcgtgagcagttcttcgggccagggacacggctcaccgtgctagaggacctgaacaaggtgttcccacccgaggtcgctgtgtttgagccatcagaagcagagatctcccacacccaaaaggccacactggtgtgcctggccacaggcttcttccccgaccacgtggagctgagctggtgggtgaatgggaaggaggtgcacagtggggtcagcacggacccgcagcccctcaaggagcagcccgccctcaatgactccagatactgcctgagcagccgcctgagggtctcggccaccttctggcagaacccccgcaaccacttccgctgtcaagtccagttctacgggctctcggagaatgacgagtggacccaggatagggccaaacccgtcacccagatcgtcagcgccgaggcctggggtagagcagactgtggctttacctcggtgtcctaccagcaaggggtcctgtctgccaccatcctctatgagatcctgctagggaaggccaccctgtatgctgtgctggtcagcgcccttgtgttgatggccatggtcaagagaaaggatttc

SEQ ID NO: 235 - DNA, 924 bp, Artificial Sequence
  Nucleotide sequence encoding TCR, Donor HD8
atgagcatcgggctcctgtgctgtgtggccttttctctcctgtgggcaagtccagtgaatgctggtgtcactcagaccccaaaattccaggtcctgaagacaggacagagcatgacactgcagtgtgcccaggatatgaaccataactccatgtactggtatcgacaagacccaggcatgggactgaggctgatttattactcagcttctgagggtaccactgacaaaggagaagtccccaatggctacaatgtctccagattaaacaaacgggagttctcgctcaggctggagtcggctgctccctcccagacatctgtgtacttctgtgccagcagggggtggcgtgagcagttcttcgggccagggacacggctcaccgtgctagaggacctgaaaaacgtgttcccacccgaggtcgctgtgtttgagccatcagaagcagagatctcccacacccaaaaggccacactggtgtgcctggccacaggcttctaccccgaccacgtggagctgagctggtgggtgaatgggaaggaggtgcacagtggggtcagcacagacccgcagcccctcaaggagcagcccgccctcaatgactccagatactgcctgagcagccgcctgagggtctcggccaccttctggcagaacccccgcaaccacttccgctgtcaagtccagttctacgggctctcggagaatgacgagtggacccaggatagggccaaacctgtcacccagatcgtcagcgccgaggcctggggtagagcagactgtggcttcacctccgagtcttaccagcaaggggtcctgtctgccaccatcctctatgagatcttgctagggaaggccaccttgtatgccgtgctggtcagtgccctcgtgctgatggccatggtcaagagaaaggattccagaggc

SEQ ID NO: 236 - DNA, 816 bp, Artificial Sequence
  Nucleotide sequence encoding TCR, Donor HD9
atggtgaagatccggcaatttttgttggctattttgtggcttcagctaagctgtgtaagtgccgccaaaaatgaagtggagcagagtcctcagaacctgactgcccaggaaggagaatttatcacaatcaactgcagttactcggtaggaataagtgccttacactggctgcaacagcatccaggaggaggcattgtttccttgtttatgctgagctcagggaagaagaagcatggaagattaattgccacaataaacatacaggaaaagcacagctccctgcacatcacagcctcccatcccagagactctgccgtctacatctgtgctgcccgatcttataacaccgacaagctcatctttgggactgggaccagattacaagtctttccaaatatccagaaccctgaccctgccgtgtaccagctgagagactctaaatccagtgacaagtctgtctgcctattcaccgattttgattctcaaacaaatgtgtcacaaagtaaggattctgatgtgtatatcacagacaaaactgtgctagacatgaggtctatggacttcaagagcaacagtgctgtggcctggagcaacaaatctgactttgcatgtgcaaacgccttcaacaacagcattattccagaagacaccttcttccccagcccagaaagttcctgtgatgtcaagctggtcgagaaaagctttgaaacagatacgaacctaaactttcaaaacctgtcagtgattgggttccgaatcctcctcctgaaagtggccgggtttaatctgctcatgacgctgcggctgtggtccagc

SEQ ID NO: 237 - DNA, 834 bp, Artificial Sequence
  Nucleotide sequence encoding TCR, Donor HD9
atggccatgctcctgggggcatcagtgctgattctgtggcttcagccagactgggtaaacagtcaacagaagaatgatgaccagcaagttaagcaaaattcaccatccctgagcgtccaggaaggaagaatttctattctgaactgtgactatactaacagcatgtttgattatttcctatggtacaaaaaataccctgctgaaggtcctacattcctgatatctataagttccattaaggataaaaatgaagatggaagattcactgtcttcttaaacaaaagtgccaagcacctctctctgcacattgtgccctcccagcctggagactctgcagtgtacttctgtgcagcaagttacaacaatgccagactcatgtttggagatggaactcagctggtggtgaagcccaatatccagaaccctgaccctgccgtgtaccagctgagagactctaaatccagtgacaagtctgtctgcctattcaccgattttgattctcaaacaaatgtgtcacaaagtaaggattctgatgtgtatatcacagacaaaactgtgctagacatgaggtctatggacttcaagagcaacagtgctgtggcctggagcaacaaatctgactttgcatgtgcaaacgccttcaacaacagcattattccagaagacaccttcttccccagcccagaaagttcctgtgatgtcaagctggtcgagaaaagctttgaaacagatacgaacctaaactttcaaaacctgtcagtgattgggttccgaatcctcctcctgaaagtggccgggtttaatctgctcatgacgctgcggctgtggtccagc

SEQ ID NO: 238 - DNA, 834 bp, Artificial Sequence; identical to SEQ ID NO: 237
  Nucleotide sequence encoding TCR, Donor HD9

SEQ ID NO: 239 - DNA, 924 bp, Artificial Sequence
  Nucleotide sequence encoding TCR, Donor HD9
atgggacccaggctcctcttctgggcactgctttgtctcctcggaacaggcccagtggaggctggagtcacacaaagtcccacacacctgatcaaaacgagaggacagcaagcgactctgagatgctctcctatctctgggcacaccagtgtgtactggtaccaacaggccctgggtctgggcctccagttcctcctttggtatgacgagggtgaagagagaaacagaggaaacttccctcctagattttcaggtcgccagttccctaattatagctctgagctgaatgtgaacgccttggagctggaggactcggccctgtatctctgtgccagcagctgggggtaccaagagacccagtacttcgggccaggcacgcggctcctggtgctcgaggacctgaacaaggtgttcccacccgaggtcgctgtgtttgagccatcagaagcagagatctcccacacccaaaaggccacactggtgtgcctggccacaggcttcttccccgaccacgtggagctgagctggtgggtgaatgggaaggaggtgcacagtggggtcagcacggacccgcagcccctcaaggagcagcccgccctcaatgactccagatactgcctgagcagccgcctgagggtctcggccaccttctggcagaacccccgcaaccacttccgctgtcaagtccagttctacgggctctcggagaatgacgagtggacccaggatagggccaaacccgtcacccagatcgtcagcgccgaggcctggggtagagcagactgtggctttacctcggtgtcctaccagcaaggggtcctgtctgccaccatcctctatgagatcctgctagggaaggccaccctgtatgctgtgctggtcagcgcccttgtgttgatggccatggtcaagagaaaggatttc

SEQ ID NO: 240 - DNA, 930 bp, Artificial Sequence
  Nucleotide sequence encoding TCR, Donor HD9
atgggacccaggctcctcttctgggcactgctttgtctcctcggaacaggcccagtggaggctggagtcacacaaagtcccacacacctgatcaaaacgagaggacagcaagcgactctgagatgctctcctatctctgggcacaccagtgtgtactggtaccaacaggccctgggtctgggcctccagttcctcctttggtatgacgagggtgaagagagaaacagaggaaacttccctcctagattttcaggtcgccagttccctaattatagctctgagctgaatgtgaacgccttggagctggaggactcggccctgtatctctgtgccagcagctgggggtaccaagagacccagtacttcgggccaggcacgcggctcctggtgctcgaggacctgaaaaacgtgttcccacccgaggtcgctgtgtttgagccatcagaagcagagatctcccacacccaaaaggccacactggtgtgcctggccacaggcttctaccccgaccacgtggagctgagctggtgggtgaatgggaaggaggtgcacagtggggtcagcacagacccgcagcccctcaaggagcagcccgccctcaatgactccagatactgcctgagcagccgcctgagggtctcggccaccttctggcagaacccccgcaaccacttccgctgtcaagtccagttctacgggctctcggagaatgacgagtggacccaggatagggccaaacctgtcacccagatcgtcagcgccgaggcctggggtagagcagactgtggcttcacctccgagtcttaccagcaaggggtcctgtctgccaccatcctctatgagatcttgctagggaaggccaccttgtatgccgtgctggtcagtgccctcgtgctgatggccatggtcaagagaaaggattccagaggc

SEQ ID NO: 241 - DNA, 933 bp, Artificial Sequence
  Nucleotide sequence encoding TCR, Donor HD9
atggacaccagagtactctgctgtgcggtcatctgtcttctgggggcaggtctctcaaatgccggcgtcatgcagaacccaagacacctggtcaggaggaggggacaggaggcaagactgagatgcagcccaatgaaaggacacagtcatgtttactggtatcggcagctcccagaggaaggtctgaaattcatggtttatctccagaaagaaaatatcatagatgagtcaggaatgccaaaggaacgattttctgctgaatttcccaaagagggccccagcatcctgaggatccagcaggtagtgcgaggagattcggcagcttatttctgtgccagctcaccgacaggtggcgagtactatggctacaccttcggttcggggaccaggttaaccgttgtagaggacctgaacaaggtgttcccacccgaggtcgctgtgtttgagccatcagaagcagagatctcccacacccaaaaggccacactggtgtgcctggccacaggcttcttccccgaccacgtggagctgagctggtgggtgaatgggaaggaggtgcacagtggggtcagcacggacccgcagcccctcaaggagcagcccgccctcaatgactccagatactgcctgagcagccgcctgagggtctcggccaccttctggcagaacccccgcaaccacttccgctgtcaagtccagttctacgggctctcggagaatgacgagtggacccaggatagggccaaacccgtcacccagatcgtcagcgccgaggcctggggtagagcagactgtggctttacctcggtgtcctaccagcaaggggtcctgtctgccaccatcctctatgagatcctgctagggaaggccaccctgtatgctgtgctggtcagcgcccttgtgttgatggccatggtcaagagaaaggatttc

SEQ ID NO: 242 - DNA, 939 bp, Artificial Sequence
  Nucleotide sequence encoding TCR, Donor HD9
atggacaccagagtactctgctgtgcggtcatctgtcttctgggggcaggtctctcaaatgccggcgtcatgcagaacccaagacacctggtcaggaggaggggacaggaggcaagactgagatgcagcccaatgaaaggacacagtcatgtttactggtatcggcagctcccagaggaaggtctgaaattcatggtttatctccagaaagaaaatatcatagatgagtcaggaatgccaaaggaacgattttctgctgaatttcccaaagagggccccagcatcctgaggatccagcaggtagtgcgaggagattcggcagcttatttctgtgccagctcaccgacaggtggcgagtactatggctacaccttcggttcggggaccaggttaaccgttgtagaggacctgaaaaacgtgttcccacccgaggtcgctgtgtttgagccatcagaagcagagatctcccacacccaaaaggccacactggtgtgcctggccacaggcttctaccccgaccacgtggagctgagctggtgggtgaatgggaaggaggtgcacagtggggtcagcacagacccgcagcccctcaaggagcagcccgccctcaatgactccagatactgcctgagcagccgcctgagggtctcggccaccttctggcagaacccccgcaaccacttccgctgtcaagtccagttctacgggctctcggagaatgacgagtggacccaggatagggccaaacctgtcacccagatcgtcagcgccgaggcctggggtagagcagactgtggcttcacctccgagtcttaccagcaaggggtcctgtctgccaccatcctctatgagatcttgctagggaaggccaccttgtatgccgtgctggtcagtgccctcgtgctgatggccatggtcaagagaaaggattccagaggc

SEQ ID NO: 243 - DNA, 954 bp, Artificial Sequence
  Nucleotide sequence encoding TCR, Donor HD9
atgagcatcggcctcctgtgctgtgcagccttgtctctcctgtgggcaggtccagtgaatgctggtgtcactcagaccccaaaattccaggtcctgaagacaggacagagcatgacactgcagtgtgcccaggatatgaaccatgaatacatgtcctggtatcgacaagacccaggcatggggctgaggctgattcattactcagttggtgctggtatcactgaccaaggagaagtccccaatggctacaatgtctccagatcaaccacagaggatttcccgctcaggctgctgtcggctgctccctcccagacatctgtgtacttctgtgccagcagttcatacccccttcggacagggcgatacaactcctataattcacccctccactttgggaacgggaccaggctcactgtgacagaggacctgaacaaggtgttcccacccgaggtcgctgtgtttgagccatcagaagcagagatctcccacacccaaaaggccacactggtgtgcctggccacaggcttcttccccgaccacgtggagctgagctggtgggtgaatgggaaggaggtgcacagtggggtcagcacggacccgcagcccctcaaggagcagcccgccctcaatgactccagatactgcctgagcagccgcctgagggtctcggccaccttctggcagaacccccgcaaccacttccgctgtcaagtccagttctacgggctctcggagaatgacgagtggacccaggatagggccaaacccgtcacccagatcgtcagcgccgaggcctggggtagagcagactgtggctttacctcggtgtcctaccagcaaggggtcctgtctgccaccatcctctatgagatcctgctagggaaggccaccctgtatgctgtgctggtcagcgcccttgtgttgatggccatggtcaagagaaaggatttctga

SEQ ID NO: 244 - DNA, 957 bp, Artificial Sequence
  Nucleotide sequence encoding TCR, Donor HD9
atgagcatcggcctcctgtgctgtgcagccttgtctctcctgtgggcaggtccagtgaatgctggtgtcactcagaccccaaaattccaggtcctgaagacaggacagagcatgacactgcagtgtgcccaggatatgaaccatgaatacatgtcctggtatcgacaagacccaggcatggggctgaggctgattcattactcagttggtgctggtatcactgaccaaggagaagtccccaatggctacaatgtctccagatcaaccacagaggatttcccgctcaggctgctgtcggctgctccctcccagacatctgtgtacttctgtgccagcagttcatacccccttcggacagggcgatacaactcctataattcacccctccactttgggaacgggaccaggctcactgtgacagaggacctgaaaaacgtgttcccacccgaggtcgctgtgtttgagccatcagaagcagagatctcccacacccaaaaggccacactggtgtgcctggccacaggcttctaccccgaccacgtggagctgagctggtgggtgaatgggaaggaggtgcacagtggggtcagcacagacccgcagcccctcaaggagcagcccgccctcaatgactccagatactgcctgagcagccgcctgagggtctcggccaccttctggcagaacccccgcaaccacttccgctgtcaagtccagttctacgggctctcggagaatgacgagtggacccaggatagggccaaacctgtcacccagatcgtcagcgccgaggcctggggtagagcagactgtggcttcacctccgagtcttaccagcaaggggtcctgtctgccaccatcctctatgagatcttgctagggaaggccaccttgtatgccgtgctggtcagtgccctcgtgctgatggccatggtcaagagaaaggattccagaggc

SEQ ID NO: 245 - DNA, 837 bp, Artificial Sequence
  Nucleotide sequence encoding TCR, Donor HD10
atggccatgctcctgggggcatcagtgctgattctgtggcttcagccagactgggtaaacagtcaacagaagaatgatgaccagcaagttaagcaaaattcaccatccctgagcgtccaggaaggaagaatttctattctgaactgtgactatactaacagcatgtttgattatttcctatggtacaaaaaataccctgctgaaggtcctacattcctgatatctataagttccattaaggataaaaatgaagatggaagattcactgtcttcttaaacaaaagtgccaagcacctctctctgcacattgtgccctcccagcctggagactctgcagtgtacttctgtgcagcaagcggaggaagagatgacaagatcatctttggaaaagggacacgacttcatattctccccaatatccagaaccctgaccctgccgtgtaccagctgagagactctaaatccagtgacaagtctgtctgcctattcaccgattttgattctcaaacaaatgtgtcacaaagtaaggattctgatgtgtatatcacagacaaaactgtgctagacatgaggtctatggacttcaagagcaacagtgctgtggcctggagcaacaaatctgactttgcatgtgcaaacgccttcaacaacagcattattccagaagacaccttcttccccagcccagaaagttcctgtgatgtcaagctggtcgagaaaagctttgaaacagatacgaacctaaactttcaaaacctgtcagtgattgggttccgaatcctcctcctgaaagtggccgggtttaatctgctcatgacgctgcggctgtggtccagc

SEQ ID NO: 246 - DNA, 933 bp, Artificial Sequence
  Nucleotide sequence encoding TCR, Donor HD10
atgagcatcggcctcctgtgctgtgcagccttgtctctcctgtgggcaggtccagtgaatgctggtgtcactcagaccccaaaattccaggtcctgaagacaggacagagcatgacactgcagtgtgcccaggatatgaaccatgaatacatgtcctggtatcgacaagacccaggcatggggctgaggctgattcattactcagttggtgctggtatcactgaccaaggagaagtccccaatggctacaatgtctccagatcaaccacagaggatttcccgctcaggctgctgtcggctgctccctcccagacatctgtgtacttctgtgccagcagctactcccggacagagagcacagatacgcagtattttggcccaggcacccggctgacagtgctcgaggacctgaacaaggtgttcccacccgaggtcgctgtgtttgagccatcagaagcagagatctcccacacccaaaaggccacactggtgtgcctggccacaggcttcttccccgaccacgtggagctgagctggtgggtgaatgggaaggaggtgcacagtggggtcagcacggacccgcagcccctcaaggagcagcccgccctcaatgactccagatactgcctgagcagccgcctgagggtctcggccaccttctggcagaacccccgcaaccacttccgctgtcaagtccagttctacgggctctcggagaatgacgagtggacccaggatagggccaaacccgtcacccagatcgtcagcgccgaggcctggggtagagcagactgtggctttacctcggtgtcctaccagcaaggggtcctgtctgccaccatcctctatgagatcctgctagggaaggccaccctgtatgctgtgctggtcagcgcccttgtgttgatggccatggtcaagagaaaggatttc

SEQ ID NO: 247 - DNA, 939 bp, Artificial Sequence
  Nucleotide sequence encoding TCR, Donor HD10
atgagcatcggcctcctgtgctgtgcagccttgtctctcctgtgggcaggtccagtgaatgctggtgtcactcagaccccaaaattccaggtcctgaagacaggacagagcatgacactgcagtgtgcccaggatatgaaccatgaatacatgtcctggtatcgacaagacccaggcatggggctgaggctgattcattactcagttggtgctggtatcactgaccaaggagaagtccccaatggctacaatgtctccagatcaaccacagaggatttcccgctcaggctgctgtcggctgctccctcccagacatctgtgtacttctgtgccagcagctactcccggacagagagcacagatacgcagtattttggcccaggcacccggctgacagtgctcgaggacctgaaaaacgtgttcccacccgaggtcgctgtgtttgagccatcagaagcagagatctcccacacccaaaaggccacactggtgtgcctggccacaggcttctaccccgaccacgtggagctgagctggtgggtgaatgggaaggaggtgcacagtggggtcagcacagacccgcagcccctcaaggagcagcccgccctcaatgactccagatactgcctgagcagccgcctgagggtctcggccaccttctggcagaacccccgcaaccacttccgctgtcaagtccagttctacgggctctcggagaatgacgagtggacccaggatagggccaaacctgtcacccagatcgtcagcgccgaggcctggggtagagcagactgtggcttcacctccgagtcttaccagcaaggggtcctgtctgccaccatcctctatgagatcttgctagggaaggccaccttgtatgccgtgctggtcagtgccctcgtgctgatggccatggtcaagagaaaggattccagaggc

SEQ ID NO: 248 - protein, 15 aa, Artificial Sequence
  WT1 peptide 91
CMTWNQMNLGATLKG

SEQ ID NO: 249 - protein, 15 aa, Artificial Sequence
  WT1 peptide 92
NQMNLGATLKGVAAG

SEQ ID NO: 250 - protein, 11 aa, Artificial Sequence
  WT1 peptide Overlapping sequence
NQMNLGATLKG

SEQ ID NO: 251 - protein, 15 aa, Artificial Sequence
  WT1 peptide 24
DPGGIWAKLGAAEAS

SEQ ID NO: 252 - protein, 15 aa, Artificial Sequence
  WT1 peptide 101
NHTTPILCGAQYRIH

SEQ ID NO: 253 - protein, 15 aa, Artificial Sequence
  WT1 peptide 125
KRHQRRHTGVKPFQC

SEQ ID NO: 254 - protein, 15 aa, Artificial Sequence
  WT1 peptide 137
PSCQKKFARSDELVR

SEQ ID NO: 255 - protein, 9 aa, Artificial Sequence
  WT1 126-134 epitope
RMFPNAPYL

SEQ ID NO: 256 - DNA, 816 bp, Artificial Sequence
  HD1a TCR sequence
atggaaaccctgctgaaggtgctgagcggcacactgctgtggcagctgacatgggtccgatctcagcagcctgtgcagtctcctcaggccgtgattctgagagaaggcgaggacgccgtgatcaactgcagcagctctaaggccctgtacagcgtgcactggtacagacagaagcacggcgaggcccctgtgttcctgatgatcctgctgaaaggcggcgagcagaagggccacgagaagatcagcgccagcttcaacgagaagaagcagcagtccagcctgtacctgacagccagccagctgagctacagcggcacctacttttgtggcaccgcctggatcaacgactacaagctgtctttcggagccggcaccacagtgacagtgcgggccaatattcagaaccccgatcctgccgtgtaccagctgagagacagcaagagcagcgacaagagcgtgtgcctgttcaccgacttcgacagccagaccaacgtgtcccagagcaaggacagcgacgtgtacatcaccgataagtgcgtgctggacatgcggagcatggacttcaagagcaacagcgccgtggcctggtccaacaagagcgatttcgcctgcgccaacgccttcaacaacagcattatccccgaggacacattcttcccaagtcctgagagcagctgcgacgtgaagctggtggaaaagagcttcgagacagacaccaacctgaacttccagaacctgagcgtgatcggcttcagaatcctgctgctcaaggtggccggcttcaacctgctgatgaccctgagactgtggtccagc

SEQ ID NO: 257 - protein, 272 aa, Artificial Sequence
  HD1a TCR sequence
METLLKVLSGTLLWQLTWVRSQQPVQSPQAVILREGEDAVINCSSSKALYSVHWYRQKHGEAPVFLMILLKGGEQKGHEKISASFNEKKQQSSLYLTASQLSYSGTYFCGTAWINDYKLSFGAGTTVTVRANIQNPDPAVYQLRDSKSSDKSVCLFTDFDSQTNVSQSKDSDVYITDKCVLDMRSMDFKSNSAVAWSNKSDFACANAFNNSIIPEDTFFPSPESSCDVKLVEKSFETDTNLNFQNLSVIGFRILLLKVAGFNLLMTLRLWSS

SEQ ID NO: 258 - DNA, 942 bp, Artificial Sequence
  HD1b TCR sequence
atgggatcttggacactgtgttgcgtgtccctgtgcatcctggtggccaagcacacagatgccggcgtgatccagtctcctagacacgaagtgaccgagatgggccaagaagtgaccctgcgctgcaagcctatcagcggccacgattacctgttctggtacagacagaccatgatgagaggcctggaactgctgatctacttcaacaacaacgtgcccatcgacgacagcggcatgcccgaggatagattcagcgccaagatgcccaacgccagcttcagcaccctgaagatccagcctagcgagcccagagatagcgccgtgtacttctgcgccagcagaaagacaggcggctacagcaatcagccccagcactttggagatggcacccggctgagcatcctggaagatctgaagaacgtgttcccacctgaggtggccgtgttcgagccttctgaggccgagatcagccacacacagaaagccacactcgtgtgtctggccaccggcttctatcccgatcacgtggaactgtcttggtgggtcaacggcaaagaggtgcacagcggcgtctgtaccgatcctcagcctctgaaagagcagcccgctctgaacgacagcagatactgcctgagcagcagactgagagtgtccgccaccttctggcagaaccccagaaaccacttcagatgccaggtgcagttctacggcctgagcgagaacgatgagtggacccaggatagagccaagcctgtgacacagatcgtgtctgccgaagcctggggcagagccgattgtggctttaccagcgagagctaccagcagggcgtgctgtctgccacaatcctgtacgagatcctgctgggcaaagccactctgtacgccgtgctggtgtctgccctggtgctgatggccatggtcaagcggaaggatagcaggggc

SEQ ID NO: 259 - protein, 314 aa, Artificial Sequence
  HD1b TCR sequence
MGSWTLCCVSLCILVAKHTDAGVIQSPRHEVTEMGQEVTLRCKPISGHDYLFWYRQTMMRGLELLIYFNNNVPIDDSGMPEDRFSAKMPNASFSTLKIQPSEPRDSAVYFCASRKTGGYSNQPQHFGDGTRLSILEDLKNVFPPEVAVFEPSEAEISHTQKATLVCLATGFYPDHVELSWWVNGKEVHSGVCTDPQPLKEQPALNDSRYCLSSRLRVSATFWQNPRNHFRCQVQFYGLSENDEWTQDRAKPVTQIVSAEAWGRADCGFTSESYQQGVLSATILYEILLGKATLYAVLVSALVLMAMVKRKDSRG

SEQ ID NO: 260 - DNA, 822 bp, Artificial Sequence
  HD3a TCR sequence
atgatcagcctgagagtgctgctggtcatcctgtggctgcagctgtcttgggtctggtcccagcggaaagaggtggaacaggaccccggacctttcaatgtgcctgaaggcgccaccgtggccttcaactgcacctacagcaatagcgccagccagagcttcttctggtacagacaggactgccggaaagaacccaagctgctgatgagcgtgtacagcagcggcaacgaggacggcagattcacagcccagctgaacagagccagccagtacatcagcctgctgatccgggatagcaagctgagcgatagcgccacctacctgtgcgtggtcaacctgctgtctaatcaaggcggcaagctgatcttcggccagggcacagagctgagcgtgaagcccaacattcagaaccccgatcctgccgtgtaccagctgagagacagcaagagcagcgacaagagcgtgtgcctgttcaccgacttcgacagccagaccaacgtgtcccagagcaaggacagcgacgtgtacatcaccgataagtgcgtgctggacatgcggagcatggacttcaagagcaacagcgccgtggcctggtccaacaagagcgatttcgcctgcgccaacgccttcaacaacagcattatccccgaggacacattcttcccaagtcctgagagcagctgcgacgtgaagctggtggaaaagagcttcgagacagacaccaacctgaacttccagaacctgtccgtgatcggcttccggatcctgctgctgaaagtggccggcttcaacctcctgatgaccctgagactgtggtccagc

SEQ ID NO: 261 - protein, 274 aa, Artificial Sequence
  HD3a TCR sequence
MISLRVLLVILWLQLSWVWSQRKEVEQDPGPFNVPEGATVAFNCTYSNSASQSFFWYRQDCRKEPKLLMSVYSSGNEDGRFTAQLNRASQYISLLIRDSKLSDSATYLCVVNLLSNQGGKLIFGQGTELSVKPNIQNPDPAVYQLRDSKSSDKSVCLFTDFDSQTNVSQSKDSDVYITDKCVLDMRSMDFKSNSAVAWSNKSDFACANAFNNSIIPEDTFFPSPESSCDVKLVEKSFETDTNLNFQNLSVIGFRILLLKVAGFNLLMTLRLWSS

SEQ ID NO: 262 - DNA, 948 bp, Artificial Sequence
  HD3b TCR sequence
atgggatgtagacttctgtgttgcgccgtgctgtgtctgcttggagctggcgaactggtgcctatggaaaccggcgtgacccagacacctagacacctggtcatgggcatgacaaacaagaaaagcctgaagtgcgagcagcacctgggccacaatgccatgtactggtacaagcagagcgccaagaaacccctggaactgatgttcgtgtacagcctggaagagagggtcgagaacaacagcgtgcccagcagattcagccctgagtgccctaatagcagccacctgtttctgcatctgcacaccctgcagcctgaggactctgccctgtatctgtgtgccagcagccaggactacctggtgtccaacgagaagctgttcttcggcagcggcacacagctgagcgtgctggaagatctgaagaacgtgttcccacctgaggtggccgtgttcgagccttctgaggccgagatcagccacacacagaaagccacactcgtgtgtctggccaccggcttctatcccgatcacgtggaactgtcttggtgggtcaacggcaaagaggtgcacagcggcgtctgtaccgatcctcagcctctgaaagagcagcccgctctgaacgacagcagatactgcctgagcagcagactgagagtgtccgccaccttctggcagaaccccagaaaccacttcagatgccaggtgcagttctacggcctgagcgagaacgatgagtggacccaggatagagccaagcctgtgacacagatcgtgtctgccgaagcctggggcagagccgattgtggctttaccagcgagagctaccagcagggcgtgctgtctgccacaatcctgtacgagatcctgctgggaaaagccactctgtacgctgtgctggtgtccgctctggtgctgatggccatggtcaagcggaaggatagcaggggc

SEQ ID NO: 263 - protein, 316 aa, Artificial Sequence
  HD3b TCR sequence
MGCRLLCCAVLCLLGAGELVPMETGVTQTPRHLVMGMTNKKSLKCEQHLGHNAMYWYKQSAKKPLELMFVYSLEERVENNSVPSRFSPECPNSSHLFLHLHTLQPEDSALYLCASSQDYLVSNEKLFFGSGTQLSVLEDLKNVFPPEVAVFEPSEAEISHTQKATLVCLATGFYPDHVELSWWVNGKEVHSGVCTDPQPLKEQPALNDSRYCLSSRLRVSATFWQNPRNHFRCQVQFYGLSENDEWTQDRAKPVTQIVSAEAWGRADCGFTSESYQQGVLSATILYEILLGKATLYAVLVSALVLMAMVKRKDSRG

SEQ ID NO: 264 - protein, 6 aa, Artificial Sequence
  TCR amino acid sequence, Donor HD6
NSMFDY

SEQ ID NO: 265 - protein, 7 aa, Artificial Sequence
  TCR amino acid sequence, Donor HD6
ISSIKDK

SEQ ID NO: 266 - protein, 12 aa, Artificial Sequence
  TCR amino acid sequence, Donor HD6
CAASATGNQFYF

SEQ ID NO: 267 - protein, 138 aa, Artificial Sequence
  TCR amino acid sequence, Donor HD6
MAMLLGASVLILWLQPDWVNSQQKNDDQQVKQNSPSLSVQEGRISILNCDYTNSMFDYFLWYKKYPAEGPTFLISISSIKDKNEDGRFTVFLNKSAKHLSLHIVPSQPGDSAVYFCAASATGNQFYFGTGTSLTVIPN

SEQ ID NO: 268 - protein, 278 aa, Artificial Sequence
  TCR amino acid sequence, Donor HD6
MAMLLGASVLILWLQPDWVNSQQKNDDQQVKQNSPSLSVQEGRISILNCDYTNSMFDYFLWYKKYPAEGPTFLISISSIKDKNEDGRFTVFLNKSAKHLSLHIVPSQPGDSAVYFCAASATGNQFYFGTGTSLTVIPNIQNPDPAVYQLRDSKSSDKSVCLFTDFDSQTNVSQSKDSDVYITDKTVLDMRSMDFKSNSAVAWSNKSDFACANAFNNSIIPEDTFFPSPESSCDVKLVEKSFETDTNLNFQNLSVIGFRILLLKVAGFNLLMTLRLWSS

SEQ ID NO: 269 - protein, 5 aa, Artificial Sequence
  TCR amino acid sequence, Donor HD6
SGHRS

SEQ ID NO: 270 - protein, 6 aa, Artificial Sequence
  TCR amino acid sequence, Donor HD6
YFSETQ

SEQ ID NO: 271 - protein, 13 aa, Artificial Sequence
  TCR amino acid sequence, Donor HD6
CASSPGQHGELFF

SEQ ID NO: 272 - protein, 132 aa, Artificial Sequence
  TCR amino acid sequence, Donor HD6
MGSRLLCWVLLCLLGAGPVKAGVTQTPRYLIKTRGQQVTLSCSPISGHRSVSWYQQTPGQGLQFLFEYFSETQRNKGNFPGRFSGRQFSNSRSEMNVSTLELGDSALYLCASSPGQHGELFFGEGSRLTVLE

SEQ ID NO: 273 - protein, 308 aa, Artificial Sequence
  TCR amino acid sequence, Donor HD6
MGSRLLCWVLLCLLGAGPVKAGVTQTPRYLIKTRGQQVTLSCSPISGHRSVSWYQQTPGQGLQFLFEYFSETQRNKGNFPGRFSGRQFSNSRSEMNVSTLELGDSALYLCASSPGQHGELFFGEGSRLTVLEDLNKVFPPEVAVFEPSEAEISHTQKATLVCLATGFFPDHVELSWWVNGKEVHSGVSTDPQPLKEQPALNDSRYCLSSRLRVSATFWQNPRNHFRCQVQFYGLSENDEWTQDRAKPVTQIVSAEAWGRADCGFTSVSYQQGVLSATILYEILLGKATLYAVLVSALVLMAMVKRKDF

SEQ ID NO: 274 - protein, 310 aa, Artificial Sequence
  TCR amino acid sequence, Donor HD6
MGSRLLCWVLLCLLGAGPVKAGVTQTPRYLIKTRGQQVTLSCSPISGHRSVSWYQQTPGQGLQFLFEYFSETQRNKGNFPGRFSGRQFSNSRSEMNVSTLELGDSALYLCASSPGQHGELFFGEGSRLTVLEDLKNVFPPEVAVFEPSEAEISHTQKATLVCLATGFYPDHVELSWWVNGKEVHSGVSTDPQPLKEQPALNDSRYCLSSRLRVSATFWQNPRNHFRCQVQFYGLSENDEWTQDRAKPVTQIVSAEAWGRADCGFTSESYQQGVLSATILYEILLGKATLYAVLVSALVLMAMVKRKDSRG

SEQ ID NO: 275 - protein, 5 aa, Artificial Sequence
  TCR amino acid sequence, Donor HD7
TSINN

SEQ ID NO: 276 - protein, 7 aa, Artificial Sequence
  TCR amino acid sequence, Donor HD7
IRSNERE

SEQ ID NO: 277 - protein, 13 aa, Artificial Sequence
  TCR amino acid sequence, Donor HD7
CATDGDSSYKLIF

SEQ ID NO: 278 - protein, 132 aa, Artificial Sequence
  TCR amino acid sequence, Donor HD7
METLLGVSLVILWLQLARVNSQQGEEDPQALSIQEGENATMNCSYKTSINNLQWYRQNSGRGLVHLILIRSNEREKHSGRLRVTLDTSKKSSSLLITASRAADTASYFCATDGDSSYKLIFGSGTRLLVRPD

SEQ ID NO: 279 - protein, 272 aa, Artificial Sequence
  TCR amino acid sequence, Donor HD7
METLLGVSLVILWLQLARVNSQQGEEDPQALSIQEGENATMNCSYKTSINNLQWYRQNSGRGLVHLILIRSNEREKHSGRLRVTLDTSKKSSSLLITASRAADTASYFCATDGDSSYKLIFGSGTRLLVRPDIQNPDPAVYQLRDSKSSDKSVCLFTDFDSQTNVSQSKDSDVYITDKTVLDMRSMDFKSNSAVAWSNKSDFACANAFNNSIIPEDTFFPSPESSCDVKLVEKSFETDTNLNFQNLSVIGFRILLLKVAGFNLLMTLRLWSS

SEQ ID NO: 280 - protein, 6 aa, Artificial Sequence
  TCR amino acid sequence, Donor HD7
DFQATT

SEQ ID NO: 281 - protein, 7 aa, Artificial Sequence
  TCR amino acid sequence, Donor HD7
SNEGSKA

SEQ ID NO: 282 - protein, 15 aa, Artificial Sequence
  TCR amino acid sequence, Donor HD7
CSARDVLTGDYGYTF

SEQ ID NO: 283 - protein, 142 aa, Artificial Sequence
  TCR amino acid sequence, Donor HD7
MLLLLLLLGPGISLLLPGSLAGSGLGAVVSQHPSWVICKSGTSVKIECRSLDFQATTMFWYRQFPKQSLMLMATSNEGSKATYEQGVEKDKFLINHASLTLSTLTVTSAHPEDSSFYICSARDVLTGDYGYTFGSGTRLTVV

SEQ ID NO: 284 - protein, 319 aa, Artificial Sequence
  TCR amino acid sequence, Donor HD7
MLLLLLLLGPGISLLLPGSLAGSGLGAVVSQHPSWVICKSGTSVKIECRSLDFQATTMFWYRQFPKQSLMLMATSNEGSKATYEQGVEKDKFLINHASLTLSTLTVTSAHPEDSSFYICSARDVLTGDYGYTFGSGTRLTVVEDLNKVFPPEVAVFEPSEAEISHTQKATLVCLATGFFPDHVELSWWVNGKEVHSGVSTDPQPLKEQPALNDSRYCLSSRLRVSATFWQNPRNHFRCQVQFYGLSENDEWTQDRAKPVTQIVSAEAWGRADCGFTSVSYQQGVLSATILYEILLGKATLYAVLVSALVLMAMVKRKDF

SEQ ID NO: 285 - protein, 321 aa, Artificial Sequence
  TCR amino acid sequence, Donor HD7
MLLLLLLLGPGISLLLPGSLAGSGLGAVVSQHPSWVICKSGTSVKIECRSLDFQATTMFWYRQFPKQSLMLMATSNEGSKATYEQGVEKDKFLINHASLTLSTLTVTSAHPEDSSFYICSARDVLTGDYGYTFGSGTRLTVVEDLKNVFPPEVAVFEPSEAEISHTQKATLVCLATGFYPDHVELSWWVNGKEVHSGVSTDPQPLKEQPALNDSRYCLSSRLRVSATFWQNPRNHFRCQVQFYGLSENDEWTQDRAKPVTQIVSAEAWGRADCGFTSESYQQGVLSATILYEILLGKATLYAVLVSALVLMAMVKRKDSRG

SEQ ID NO: 286 - protein, 5 aa, Artificial Sequence
  TCR amino acid sequence, Donor HD7
SGHDY

SEQ ID NO: 287 - protein, 6 aa, Artificial Sequence
  TCR amino acid sequence, Donor HD7
FNNNVP

SEQ ID NO: 288 - protein, 16 aa, Artificial Sequence
  TCR amino acid sequence, Donor HD7
CASSLGLSISQETQYF

SEQ ID NO: 289 - protein, 136 aa, Artificial Sequence
  TCR amino acid sequence, Donor HD7
MGSWTLCCVSLCILVAKHTDAGVIQSPRHEVTEMGQEVTLRCKPISGHDYLFWYRQTMMRGLELLIYFNNNVPIDDSGMPEDRFSAKMPNASFSTLKIQPSEPRDSAVYFCASSLGLSISQETQYFGPGTRLLVLE

SEQ ID NO: 290 - protein, 312 aa, Artificial Sequence
  TCR amino acid sequence, Donor HD7
MGSWTLCCVSLCILVAKHTDAGVIQSPRHEVTEMGQEVTLRCKPISGHDYLFWYRQTMMRGLELLIYFNNNVPIDDSGMPEDRFSAKMPNASFSTLKIQPSEPRDSAVYFCASSLGLSISQETQYFGPGTRLLVLEDLNKVFPPEVAVFEPSEAEISHTQKATLVCLATGFFPDHVELSWWVNGKEVHSGVSTDPQPLKEQPALNDSRYCLSSRLRVSATFWQNPRNHFRCQVQFYGLSENDEWTQDRAKPVTQIVSAEAWGRADCGFTSVSYQQGVLSATILYEILLGKATLYAVLVSALVLMAMVKRKDF

SEQ ID NO: 291 - protein, 314 aa, Artificial Sequence
  TCR amino acid sequence, Donor HD7
MGSWTLCCVSLCILVAKHTDAGVIQSPRHEVTEMGQEVTLRCKPISGHDYLFWYRQTMMRGLELLIYFNNNVPIDDSGMPEDRFSAKMPNASFSTLKIQPSEPRDSAVYFCASSLGLSISQETQYFGPGTRLLVLEDLKNVFPPEVAVFEPSEAEISHTQKATLVCLATGFYPDHVELSWWVNGKEVHSGVSTDPQPLKEQPALNDSRYCLSSRLRVSATFWQNPRNHFRCQVQFYGLSENDEWTQDRAKPVTQIVSAEAWGRADCGFTSESYQQGVLSATILYEILLGKATLYAVLVSALVLMAMVKRKDSRG

SEQ ID NO: 292 - DNA, 837 bp, Artificial Sequence
  Nucleotide sequence encoding TCR, Donor HD6
atggccatgctcctgggggcatcagtgctgattctgtggcttcagccagactgggtaaacagtcaacagaagaatgatgaccagcaagttaagcaaaattcaccatccctgagcgtccaggaaggaagaatttctattctgaactgtgactatactaacagcatgtttgattatttcctatggtacaaaaaataccctgctgaaggtcctacattcctgatatctataagttccattaaggataaaaatgaagatggaagattcactgtcttcttaaacaaaagtgccaagcacctctctctgcacattgtgccctcccagcctggagactctgcagtgtacttctgtgcagcaagcgctaccggtaaccagttctattttgggacagggacaagtttgacggtcattccaaatatccagaaccctgaccctgccgtgtaccagctgagagactctaaatccagtgacaagtctgtctgcctattcaccgattttgattctcaaacaaatgtgtcacaaagtaaggattctgatgtgtatatcacagacaaaactgtgctagacatgaggtctatggacttcaagagcaacagtgctgtggcctggagcaacaaatctgactttgcatgtgcaaacgccttcaacaacagcattattccagaagacaccttcttccccagcccagaaagttcctgtgatgtcaagctggtcgagaaaagctttgaaacagatacgaacctaaactttcaaaacctgtcagtgattgggttccgaatcctcctcctgaaagtggccgggtttaatctgctcatgacgctgcggctgtggtccagctga

SEQ ID NO: 293 - DNA, 924 bp, Artificial Sequence
  Nucleotide sequence encoding TCR, Donor HD6
atgggctccaggctgctctgttgggtgctgctttgtctcctgggagcaggcccagtaaaggctggagtcactcaaactccaagatatctgatcaaaacgagaggacagcaagtgacactgagctgctcccctatctctgggcataggagtgtatcctggtaccaacagaccccaggacagggccttcagttcctctttgaatacttcagtgagacacagagaaacaaaggaaacttccctggtcgattctcagggcgccagttctctaactctcgctctgagatgaatgtgagcaccttggagctgggggactcggccctttatctttgcgccagcagccctggacagcacggggagctgttttttggagaaggctctaggctgaccgtactggaggacctgaacaaggtgttcccacccgaggtcgctgtgtttgagccatcagaagcagagatctcccacacccaaaaggccacactggtgtgcctggccacaggcttcttccccgaccacgtggagctgagctggtgggtgaatgggaaggaggtgcacagtggggtcagcacggacccgcagcccctcaaggagcagcccgccctcaatgactccagatactgcctgagcagccgcctgagggtctcggccaccttctggcagaacccccgcaaccacttccgctgtcaagtccagttctacgggctctcggagaatgacgagtggacccaggatagggccaaacccgtcacccagatcgtcagcgccgaggcctggggtagagcagactgtggctttacctcggtgtcctaccagcaaggggtcctgtctgccaccatcctctatgagatcctgctagggaaggccaccctgtatgctgtgctggtcagcgcccttgtgttgatggccatggtcaagagaaaggatttc

SEQ ID NO: 294 - DNA, 930 bp, Artificial Sequence
  Nucleotide sequence encoding TCR, Donor HD6
atgggctccaggctgctctgttgggtgctgctttgtctcctgggagcaggcccagtaaaggctggagtcactcaaactccaagatatctgatcaaaacgagaggacagcaagtgacactgagctgctcccctatctctgggcataggagtgtatcctggtaccaacagaccccaggacagggccttcagttcctctttgaatacttcagtgagacacagagaaacaaaggaaacttccctggtcgattctcagggcgccagttctctaactctcgctctgagatgaatgtgagcaccttggagctgggggactcggccctttatctttgcgccagcagccctggacagcacggggagctgttttttggagaaggctctaggctgaccgtactggaggacctgaaaaacgtgttcccacccgaggtcgctgtgtttgagccatcagaagcagagatctcccacacccaaaaggccacactggtgtgcctggccacaggcttctaccccgaccacgtggagctgagctggtgggtgaatgggaaggaggtgcacagtggggtcagcacagacccgcagcccctcaaggagcagcccgccctcaatgactccagatactgcctgagcagccgcctgagggtctcggccaccttctggcagaacccccgcaaccacttccgctgtcaagtccagttctacgggctctcggagaatgacgagtggacccaggatagggccaaacctgtcacccagatcgtcagcgccgaggcctggggtagagcagactgtggcttcacctccgagtcttaccagcaaggggtcctgtctgccaccatcctctatgagatcttgctagggaaggccaccttgtatgccgtgctggtcagtgccctcgtgctgatggccatggtcaagagaaaggattccagaggc

SEQ ID NO: 295 - DNA, 816 bp, Artificial Sequence
  Nucleotide sequence encoding TCR, Donor HD7
atggaaactctcctgggagtgtctttggtgattctatggcttcaactggctagggtgaacagtcaacagggagaagaggatcctcaggccttgagcatccaggagggtgaaaatgccaccatgaactgcagttacaaaactagtataaacaatttacagtggtatagacaaaattcaggtagaggccttgtccacctaattttaatacgttcaaatgaaagagagaaacacagtggaagattaagagtcacgcttgacacttccaagaaaagcagttccttgttgatcacggcttcccgggcagcagacactgcttcttacttctgtgctacggacggggatagcagctataaattgatcttcgggagtgggaccagactgctggtcaggcctgatatccagaaccctgaccctgccgtgtaccagctgagagactctaaatccagtgacaagtctgtctgcctattcaccgattttgattctcaaacaaatgtgtcacaaagtaaggattctgatgtgtatatcacagacaaaactgtgctagacatgaggtctatggacttcaagagcaacagtgctgtggcctggagcaacaaatctgactttgcatgtgcaaacgccttcaacaacagcattattccagaagacaccttcttccccagcccagaaagttcctgtgatgtcaagctggtcgagaaaagctttgaaacagatacgaacctaaactttcaaaacctgtcagtgattgggttccgaatcctcctcctgaaagtggccgggtttaatctgctcatgacgctgcggctgtggtccagc

SEQ ID NO: 296 - DNA, 957 bp, Artificial Sequence
  Nucleotide sequence encoding TCR, Donor HD7
atgctgctgcttctgctgcttctggggccaggtataagcctccttctacctgggagcttggcaggctccgggcttggtgctgtcgtctctcaacatccgagctgggttatctgtaagagtggaacctctgtgaagatcgagtgccgttccctggactttcaggccacaactatgttttggtatcgtcagttcccgaaacagagtctcatgctgatggcaacttccaatgagggctccaaggccacatacgagcaaggcgtcgagaaggacaagtttctcatcaaccatgcaagcctgaccttgtccactctgacagtgaccagtgcccatcctgaagacagcagcttctacatctgcagtgctagagacgtactgacaggggactatggctacaccttcggttcggggaccaggttaaccgttgtagaggacctgaacaaggtgttcccacccgaggtcgctgtgtttgagccatcagaagcagagatctcccacacccaaaaggccacactggtgtgcctggccacaggcttcttccccgaccacgtggagctgagctggtgggtgaatgggaaggaggtgcacagtggggtcagcacggacccgcagcccctcaaggagcagcccgccctcaatgactccagatactgcctgagcagccgcctgagggtctcggccaccttctggcagaacccccgcaaccacttccgctgtcaagtccagttctacgggctctcggagaatgacgagtggacccaggatagggccaaacccgtcacccagatcgtcagcgccgaggcctggggtagagcagactgtggctttacctcggtgtcctaccagcaaggggtcctgtctgccaccatcctctatgagatcctgctagggaaggccaccctgtatgctgtgctggtcagcgcccttgtgttgatggccatggtcaagagaaaggatttc

SEQ ID NO: 297 - DNA, 963 bp, Artificial Sequence
  Nucleotide sequence encoding TCR, Donor HD7
atgctgctgcttctgctgcttctggggccaggtataagcctccttctacctgggagcttggcaggctccgggcttggtgctgtcgtctctcaacatccgagctgggttatctgtaagagtggaacctctgtgaagatcgagtgccgttccctggactttcaggccacaactatgttttggtatcgtcagttcccgaaacagagtctcatgctgatggcaacttccaatgagggctccaaggccacatacgagcaaggcgtcgagaaggacaagtttctcatcaaccatgcaagcctgaccttgtccactctgacagtgaccagtgcccatcctgaagacagcagcttctacatctgcagtgctagagacgtactgacaggggactatggctacaccttcggttcggggaccaggttaaccgttgtagaggacctgaaaaacgtgttcccacccgaggtcgctgtgtttgagccatcagaagcagagatctcccacacccaaaaggccacactggtgtgcctggccacaggcttctaccccgaccacgtggagctgagctggtgggtgaatgggaaggaggtgcacagtggggtcagcacagacccgcagcccctcaaggagcagcccgccctcaatgactccagatactgcctgagcagccgcctgagggtctcggccaccttctggcagaacccccgcaaccacttccgctgtcaagtccagttctacgggctctcggagaatgacgagtggacccaggatagggccaaacctgtcacccagatcgtcagcgccgaggcctggggtagagcagactgtggcttcacctccgagtcttaccagcaaggggtcctgtctgccaccatcctctatgagatcttgctagggaaggccaccttgtatgccgtgctggtcagtgccctcgtgctgatggccatggtcaagagaaaggattccagaggc

SEQ ID NO: 298 - DNA, 936 bp, Artificial Sequence
  Nucleotide sequence encoding TCR, Donor HD7
atgggctcctggaccctctgctgtgtgtccctttgcatcctggtagcaaagcacacagatgctggagttatccagtcaccccggcacgaggtgacagagatgggacaagaagtgactctgagatgtaaaccaatttcaggacacgactaccttttctggtacagacagaccatgatgcggggactggagttgctcatttactttaacaacaacgttccgatagatgattcagggatgcccgaggatcgattctcagctaagatgcctaatgcatcattctccactctgaagatccagccctcagaacccagggactcagctgtgtacttctgtgccagcagtttaggactgagcatttcccaagagacccagtacttcgggccaggcacgcggctcctggtgctcgaggacctgaacaaggtgttcccacccgaggtcgctgtgtttgagccatcagaagcagagatctcccacacccaaaaggccacactggtgtgcctggccacaggcttcttccccgaccacgtggagctgagctggtgggtgaatgggaaggaggtgcacagtggggtcagcacggacccgcagcccctcaaggagcagcccgccctcaatgactccagatactgcctgagcagccgcctgagggtctcggccaccttctggcagaacccccgcaaccacttccgctgtcaagtccagttctacgggctctcggagaatgacgagtggacccaggatagggccaaacccgtcacccagatcgtcagcgccgaggcctggggtagagcagactgtggctttacctcggtgtcctaccagcaaggggtcctgtctgccaccatcctctatgagatcctgctagggaaggccaccctgtatgctgtgctggtcagcgcccttgtgttgatggccatggtcaagagaaaggatttc

SEQ ID NO: 299 - DNA, 942 bp, Artificial Sequence
  Nucleotide sequence encoding TCR, Donor HD7
atgggctcctggaccctctgctgtgtgtccctttgcatcctggtagcaaagcacacagatgctggagttatccagtcaccccggcacgaggtgacagagatgggacaagaagtgactctgagatgtaaaccaatttcaggacacgactaccttttctggtacagacagaccatgatgcggggactggagttgctcatttactttaacaacaacgttccgatagatgattcagggatgcccgaggatcgattctcagctaagatgcctaatgcatcattctccactctgaagatccagccctcagaacccagggactcagctgtgtacttctgtgccagcagtttaggactgagcatttcccaagagacccagtacttcgggccaggcacgcggctcctggtgctcgaggacctgaaaaacgtgttcccacccgaggtcgctgtgtttgagccatcagaagcagagatctcccacacccaaaaggccacactggtgtgcctggccacaggcttctaccccgaccacgtggagctgagctggtgggtgaatgggaaggaggtgcacagtggggtcagcacagacccgcagcccctcaaggagcagcccgccctcaatgactccagatactgcctgagcagccgcctgagggtctcggccaccttctggcagaacccccgcaaccacttccgctgtcaagtccagttctacgggctctcggagaatgacgagtggacccaggatagggccaaacctgtcacccagatcgtcagcgccgaggcctggggtagagcagactgtggcttcacctccgagtcttaccagcaaggggtcctgtctgccaccatcctctatgagatcttgctagggaaggccaccttgtatgccgtgctggtcagtgccctcgtgctgatggccatggtcaagagaaaggattccagaggc